European Patent Application EP 4 711 461 A1, published March 18, 2026. Title: 一种携带SMN基因表达框的病毒载体及其用途. Applicant: 上海金珂博生物技术有限公司. Application WO. The sequence listing filed with the application follows.

SEQUENCE LISTING (39 sequences)

SEQ ID NO: 1 - DNA, 885 bp, synthetic construct
  source 1..885: mol_type = other DNA
atggccatgtctagtggcggatctggtggcggagtgcccgagcaagaagatagcgtcctgttcagaagaggcaccggccagagcgacgacagcgacatctgggatgatacagccctgatcaaggcctacgacaaggccgtggccagctttaagcacgccctgaagaacggcgatatctgcgagacaagcggcaagcccaagaccacacctaagagaaagcccgccaagaagaacaagagccagaagaagaataccgccgccagcctgcagcagtggaaagtgggcgataagtgcagcgccatttggagcgaggacggctgtatctaccctgccacaatcgccagcatcgacttcaagcgggaaacctgcgtggtggtgtacacaggctacggcaacagagaggaacagaacctgagcgacctgctgagcccaatttgcgaggtggccaacaacatcgagcagaacgcccaagagaacgagaacgagtcccaggtgtccaccgacgagagcgagaatagcagaagccccggcaacaagagcgacaacatcaagcctaagagcgccccttggaacagcttcctgcctcctcctccaccaatgcctggacctagactcggacctggaaagcccggcctgaagttcaatggacctccaccaccgccaccacctccgcctccacatcttctgtcttgttggctgcctccatttcctagcggccctccaatcatcccgccacctccacctatctgccccgacagtctggatgatgctgatgccctgggctccatgctgatctcttggtacatgagcggctaccacaccggctactacatgggcttcagacagaaccagaaagagggccgttgcagccacagcctgaactga

SEQ ID NO: 2 - DNA, 885 bp, synthetic construct
  source 1..885: mol_type = other DNA
atggcaatgtcatcaggtggaagtggtggaggggtccctgaacaagaagacagcgtgttgtttaggcgcggcaccggacagagcgacgattctgatatctgggatgataccgcacttatcaaagcgtacgataaagctgttgcatcctttaagcacgctctcaagaacggagacatctgtgaaacgagcggcaagccaaagaccacccccaaaaggaagccagccaagaaaaataaatctcagaaaaaaaacaccgctgcaagccttcagcagtggaaggtcggtgataagtgcagcgccatttggagtgaggatggctgtatctatcctgccacaatcgcctctattgacttcaagcgcgaaacttgcgtggtagtgtataccggatatggcaatagagaggagcagaacctgtctgacctgctcagtccaatttgtgaggtcgcaaacaatattgagcagaacgcgcaggaaaatgaaaatgaatctcaggtcagcaccgatgagagcgagaattcaaggtctcccgggaataaatcagacaacatcaagcccaagtccgccccatggaattcctttttgccacctcctcctccgatgccaggacctagactgggaccaggtaaacctggtctgaagttcaatggacctcctccacctcctcctcctccaccaccacatcttctgagttgctggctgcccccctttccttctggtccccctataatccccccacctcctcccatatgccctgacagcctggatgacgccgatgccctgggaagtatgctgattagctggtacatgagcgggtaccacactggatactatatggggtttagacagaaccagaaggagggcagatgttctcactctctgaattga

SEQ ID NO: 3 - DNA, 885 bp, synthetic construct
  source 1..885: mol_type = other DNA
atggctatgtctagtggtggatctggtggcggcgtgcccgagcaagaagatagcgtcctgttcagaagaggcaccggccagagcgacgacagcgacatctgggatgatacagccctgatcaaggcctacgacaaggccgtggccagctttaagcacgccctgaagaacggcgatatctgcgagacaagcggcaagcccaagaccacacctaagagaaagcccgccaagaagaacaagagccagaagaagaataccgccgccagcctgcagcagtggaaagtgggcgataagtgcagcgccatttggagcgaggacggctgtatctaccctgccacaatcgccagcatcgacttcaagcgggaaacctgcgtggtggtgtacacaggctacggcaacagagaggaacagaacctgagcgacctgctgagcccaatttgcgaggtggccaacaacatcgagcagaacgcccaagagaacgagaacgagtcccaggtgtccaccgacgagagcgagaatagcagaagccccggcaacaagagcgacaacatcaagcctaagagcgccccttggaacagcttcctgcctcctcctccaccaatgcctggacctagactcggacctggaaagcccggcctgaagttcaatggacctccaccaccgccaccacctccgcctccacatcttctgtcttgttggctgcctccatttcctagcggccctccaatcatcccgccacctccacctatctgccccgacagtctggatgatgctgatgccctgggctccatgctgatctcttggtacatgagcggctaccacaccggctactacatgggcttcagacagaaccagaaagagggccgttgcagccacagcctgaactga

SEQ ID NO: 4 - DNA, 17 bp, synthetic construct
  source 1..17: mol_type = other DNA
taggtcaatgagggatg

SEQ ID NO: 5 - DNA, 17 bp, synthetic construct
  source 1..17: mol_type = other DNA
acttgggagtcctatga

SEQ ID NO: 6 - DNA, 17 bp, synthetic construct
  source 1..17: mol_type = other DNA
agactgatgtaaactag

SEQ ID NO: 7 - DNA, 139 bp, synthetic construct
  source 1..139: mol_type = other DNA
agtgaattctaccagtgccatataggtcaatgagggatgcaaacaccattgtcacactccaacttgggagtcctatgaagtgaattctaccagtgccataagactgatgtaaactagcaaacaccattgtcacactcca

SEQ ID NO: 8 - DNA, 885 bp, synthetic construct
  source 1..885: mol_type = other DNA
atggcgatgagcagcggcggcagtggtggcggcgtcccggagcaggaggattccgtgctgttccggcgcggcacaggccagagcgatgattctgacatttgggatgatacagcactgataaaagcatatgataaagctgtggcttcatttaagcatgctctaaagaatggtgacatttgtgaaacttcgggtaaaccaaaaaccacacctaaaagaaaacctgctaagaagaataaaagccaaaagaagaatactgcagcttccttacaacagtggaaagttggggacaaatgttctgccatttggtcagaagacggttgcatttacccagctaccattgcttcaattgattttaagagagaaacctgtgttgtggtttacactggatatggaaatagagaggagcaaaatctgtccgatctactttccccaatctgtgaagtagctaataatatagaacaaaatgctcaagagaatgaaaatgaaagccaagtttcaacagatgaaagtgagaactccaggtctcctggaaataaatcagataacatcaagcccaaatctgctccatggaactcttttctccctccaccaccccccatgccagggccaagactgggaccaggaaagccaggtctaaaattcaatggcccaccaccgccaccgccaccaccaccaccccacttactatcatgctggctgcctccatttccttctggaccaccaataattcccccaccacctcccatatgtccagattctcttgatgatgctgatgctttgggaagtatgttaatttcatggtacatgagtggctatcatactggctattatatgggttttagacaaaatcaaaaagaaggaaggtgctcacattccttaaattaa

SEQ ID NO: 9 - DNA, 5910 bp, synthetic construct
  source 1..5910: mol_type = other DNA
ctgcgcgctcgctcgctcactgaggccgcccgggcaaagcccgggcgtcgggcgacctttggtcgcccggcctcagtgagcgagcgagcgcgcagagagggagtggaattcacgcgtggatctgaattcaattcacgcgtggtacctctggtcgttacataacttacggtaaatggcccgcctggctgaccgcccaacgacccccgcccattgacgtcaataatgacgtatgttcccatagtaacgccaatagggactttccattgacgtcaatgggtggagtatttacggtaaactgcccacttggcagtacatcaagtgtatcatatgccaagtacgccccctattgacgtcaatgacggtaaatggcccgcctggcattatgcccagtacatgaccttatgggactttcctacttggcagtacatctactcgaggccacgttctgcttcactctccccatctcccccccctccccacccccaattttgtatttatttattttttaattattttgtgcagcgatgggggcggggggggggggggggcgcgcgccaggcggggcggggcggggcgaggggcggggcggggcgaggcggagaggtgcggcggcagccaatcagagcggcgcgctccgaaagtttccttttatggcgaggcggcggcggcggcggccctataaaaagcgaagcgcgcggcgggcgggagcgggatcagccaccgcggtggcggcctagagtcgacgaggaactgaaaaaccagaaagttaactggtaagtttagtctttttgtcttttatttcaggtcccggatccggtggtggtgcaaatcaaagaactgctcctcagtggatgttgcctttacttctaggcctgtacggaagtgttacttctgctctaaaagctgcggaattgtacccgcggccgatccaccggtccggaattcccgggatatcgtcgacccacgcgtccgggcccatggcgatgagcagcggcggcagtggtggcggcgtcccggagcaggaggattccgtgctgttccggcgcggcacaggccagagcgatgattctgacatttgggatgatacagcactgataaaagcatatgataaagctgtggcttcatttaagcatgctctaaagaatggtgacatttgtgaaacttcgggtaaaccaaaaaccacacctaaaagaaaacctgctaagaagaataaaagccaaaagaagaatactgcagcttccttacaacagtggaaagttggggacaaatgttctgccatttggtcagaagacggttgcatttacccagctaccattgcttcaattgattttaagagagaaacctgtgttgtggtttacactggatatggaaatagagaggagcaaaatctgtccgatctactttccccaatctgtgaagtagctaataatatagaacaaaatgctcaagagaatgaaaatgaaagccaagtttcaacagatgaaagtgagaactccaggtctcctggaaataaatcagataacatcaagcccaaatctgctccatggaactcttttctccctccaccaccccccatgccagggccaagactgggaccaggaaagccaggtctaaaattcaatggcccaccaccgccaccgccaccaccaccaccccacttactatcatgctggctgcctccatttccttctggaccaccaataattcccccaccacctcccatatgtccagattctcttgatgatgctgatgctttgggaagtatgttaatttcatggtacatgagtggctatcatactggctattatatgggttttagacaaaatcaaaaagaaggaaggtgctcacattccttaaattaaagatctagaaagcttatcgataccgtcgactagagctcgctgatcagcctcgactgtgccttctagttgccagccatctgttgtttgcccctcccccgtgccttccttgaccctggaaggtgccactcccactgtcctttcctaataaaatgaggaaattgcatcgcattgtctgagtaggtgtcattctattctggggggtggggtggggcaggacagcaagggggaggattgggaagacaatagcaggcatgctggggagagatcgatctgaggaacccctagtgatggagttggccactccctctctgcgcgctcgctcgctcactgaggccgggcgaccaaaggtcgcccgacgcccgggctttgcccgggcggcctcagtgagcgagcgagcgcgcagagagggagtggcccccccccccccccccccggcgattctcttgtttgctccagactctcaggcaatgacctgatagcctttgtagagacctctcaaaaatagctaccctctccggcatgaatttatcagctagaacggttgaatatcatattgatggtgatttgactgtctccggcctttctcacccgtttgaatctttacctacacattactcaggcattgcatttaaaatatatgagggttctaaaaatttttatccttgcgttgaaataaaggcttctcccgcaaaagtattacagggtcataatgtttttggtacaaccgatttagctttatgctctgaggctttattgcttaattttgctaattctttgccttgcctgtatgatttattggatgttggaatcgcctgatgcggtattttctccttacgcatctgtgcggtatttcacaccgcatatggtgcactctcagtacaatctgctctgatgccgcatagttaagccagccccgacacccgccaacactatggtgcactctcagtacaatctgctctgatgccgcatagttaagccagccccgacacccgccaacacccgctgacgcgccctgacgggcttgtctgctcccggcatccgcttacagacaagctgtgaccgtctccgggagctgcatgtgtcagaggttttcaccgtcatcaccgaaacgcgcgagacgaaagggcctcgtgatacgcctatttttataggttaatgtcatgataataatggtttcttagacgtcaggtggcacttttcggggaaatgtgcgcggaacccctatttgtttatttttctaaatacattcaaatatgtatccgctcatgagacaataaccctgataaatgcttcaataatattgaaaaaggaagagtatgagccatattcaacgggaaacgtcgaggccgcgattaaattccaacatggatgctgatttatatgggtataaatgggctcgcgataatgtcgggcaatcaggtgcgacaatctatcgcttgtatgggaagcccgatgcgccagagttgtttctgaaacatggcaaaggtagcgttgccaatgatgttacagatgagatggtcagactaaactggctgacggaatttatgccacttccgaccatcaagcattttatccgtactcctgatgatgcatggttactcaccactgcgatccccggaaaaacagcgttccaggtattagaagaatatcctgattcaggtgaaaatattgttgatgcgctggcagtgttcctgcgccggttgcactcgattcctgtttgtaattgtccttttaacagcgatcgcgtatttcgcctcgctcaggcgcaatcacgaatgaataacggtttggttgatgcgagtgattttgatgacgagcgtaatggctggcctgttgaacaagtctggaaagaaatgcataaacttttgccattctcaccggattcagtcgtcactcatggtgatttctcacttgataaccttatttttgacgaggggaaattaataggttgtattgatgttggacgagtcggaatcgcagaccgataccaggatcttgccatcctatggaactgcctcggtgagttttctccttcattacagaaacggctttttcaaaaatatggtattgataatcctgatatgaataaattgcagtttcatttgatgctcgatgagtttttctaactgtcagaccaagtttactcatatatactttagattgatttaaaacttcatttttaatttaaaaggatctaggtgaagatcctttttgataatctcatgaccaaaatcccttaacgtgagttttcgttccactgagcgtcagaccccgtagaaaagatcaaaggatcttcttgagatcctttttttctgcgcgtaatctgctgcttgcaaacaaaaaaaccaccgctaccagcggtggtttgtttgccggatcaagagctaccaactctttttccgaaggtaactggcttcagcagagcgcagataccaaatactgttcttctagtgtagccgtagttaggccaccacttcaagaactctgtagcaccgcctacatacctcgctctgctaatcctgttaccagtggctgctgccagtggcgataagtcgtgtcttaccgggttggactcaagacgatagttaccggataaggcgcagcggtcgggctgaacggggggttcgtgcacacagcccagcttggagcgaacgacctacaccgaactgagatacctacagcgtgagctatgagaaagcgccacgcttcccgaagggagaaaggcggacaggtatccggtaagcggcagggtcggaacaggagagcgcacgagggagcttccagggggaaacgcctggtatctttatagtcctgtcgggtttcgccacctctgacttgagcgtcgatttttgtgatgctcgtcaggggggcggagcctatggaaaaacgccagcaacgcggcctttttacggttcctggccttttgctggccttttgctcacatgttctttcctgcgttatcccctgattctgtggataaccgtattaccgcctttgagtgagctgataccgctcgccgcagccgaacgaccgagcgcagcgagtcagtgagcgaggaagcggaagagcgcccaatacgcaaaccgcctctccccgcgcgttggccgattcattaatgcagctggcgtaatagcgaagaggcccgcaccgatcgcccttcccaacagttgcgcagcctgaatggcgaatggcgattccgttgcaatggctggcggtaatattgttctggatattaccagcaaggccgatagtttgagttcttctactcaggcaagtgatgttattactaatcaaagaagtattgcgacaacggttaatttgcgtgatggacagactcttttactcggtggcctcactgattataaaaacacttctcaggattctggcgtaccgttcctgtctaaaatccctttaatcggcctcctgtttagctcccgctctgattctaacgaggaaagcacgttatacgtgctcgtcaaagcaaccatagtacgcgccctgtagcggcgcattaagcgcggcgggtgtggtggttacgcgcagcgtgaccgctacacttgccagcgccctagcgcccgctcctttcgctttcttcccttcctttctcgccacgttcgccggctttccccgtcaagctctaaatcgggggctccctttagggttccgatttagtgctttacggcacctcgaccccaaaaaacttgattagggtgatggttcacgtagtgggccatcgccctgatagacggtttttcgccctttgacgttggagtccacgttctttaatagtggactcttgttccaaactggaacaacactcaaccctatctcggtctattcttttgatttataagggattttgccgatttcggcctattggttaaaaaatgagctgatttaacaaaaatttaacgcgaattttaacaaaatattaacgcttacaatttaaatatttgcttatacaatcttcctgtttttggggcttttctgattatcaaccggggtacatatgattgacatgctagttttacgattaccgttcatcgcc

SEQ ID NO: 10 - DNA, 5935 bp, synthetic construct
  source 1..5935: mol_type = other DNA
ctgcgcgctcgctcgctcactgaggccgcccgggcaaagcccgggcgtcgggcgacctttggtcgcccggcctcagtgagcgagcgagcgcgcagagagggagtggaattcacgcgtggatctgaattcaattcacgcgtggtacctctggtcgttacataacttacggtaaatggcccgcctggctgaccgcccaacgacccccgcccattgacgtcaataatgacgtatgttcccatagtaacgccaatagggactttccattgacgtcaatgggtggagtatttacggtaaactgcccacttggcagtacatcaagtgtatcatatgccaagtacgccccctattgacgtcaatgacggtaaatggcccgcctggcattatgcccagtacatgaccttatgggactttcctacttggcagtacatctactcgaggccacgttctgcttcactctccccatctcccccccctccccacccccaattttgtatttatttattttttaattattttgtgcagcgatgggggcggggggggggggggggcgcgcgccaggcggggcggggcggggcgaggggcggggcggggcgaggcggagaggtgcggcggcagccaatcagagcggcgcgctccgaaagtttccttttatggcgaggcggcggcggcggcggccctataaaaagcgaagcgcgcggcgggcgggagcgggatcagccaccgcggtggcggcctagagtcgacgaggaactgaaaaaccagaaagttaactggtaagtttagtctttttgtcttttatttcaggtcccggatccggtggtggtgcaaatcaaagaactgctcctcagtggatgttgcctttacttctaggcctgtacggaagtgttacttctgctctaaaagctgcggaattgtacccgcggccgatccaccggtccggaattcccgggatatcgtcgacccacgcgtccgggccccacgctgcgcacccgcgggtttgctatggccatgtctagtggcggatctggtggcggagtgcccgagcaagaagatagcgtcctgttcagaagaggcaccggccagagcgacgacagcgacatctgggatgatacagccctgatcaaggcctacgacaaggccgtggccagctttaagcacgccctgaagaacggcgatatctgcgagacaagcggcaagcccaagaccacacctaagagaaagcccgccaagaagaacaagagccagaagaagaataccgccgccagcctgcagcagtggaaagtgggcgataagtgcagcgccatttggagcgaggacggctgtatctaccctgccacaatcgccagcatcgacttcaagcgggaaacctgcgtggtggtgtacacaggctacggcaacagagaggaacagaacctgagcgacctgctgagcccaatttgcgaggtggccaacaacatcgagcagaacgcccaagagaacgagaacgagtcccaggtgtccaccgacgagagcgagaatagcagaagccccggcaacaagagcgacaacatcaagcctaagagcgccccttggaacagcttcctgcctcctcctccaccaatgcctggacctagactcggacctggaaagcccggcctgaagttcaatggacctccaccaccgccaccacctccgcctccacatcttctgtcttgttggctgcctccatttcctagcggccctccaatcatcccgccacctccacctatctgccccgacagtctggatgatgctgatgccctgggctccatgctgatctcttggtacatgagcggctaccacaccggctactacatgggcttcagacagaaccagaaagagggccgttgcagccacagcctgaactgaagatctagaaagcttatcgataccgtcgactagagctcgctgatcagcctcgactgtgccttctagttgccagccatctgttgtttgcccctcccccgtgccttccttgaccctggaaggtgccactcccactgtcctttcctaataaaatgaggaaattgcatcgcattgtctgagtaggtgtcattctattctggggggtggggtggggcaggacagcaagggggaggattgggaagacaatagcaggcatgctggggagagatcgatctgaggaacccctagtgatggagttggccactccctctctgcgcgctcgctcgctcactgaggccgggcgaccaaaggtcgcccgacgcccgggctttgcccgggcggcctcagtgagcgagcgagcgcgcagagagggagtggcccccccccccccccccccggcgattctcttgtttgctccagactctcaggcaatgacctgatagcctttgtagagacctctcaaaaatagctaccctctccggcatgaatttatcagctagaacggttgaatatcatattgatggtgatttgactgtctccggcctttctcacccgtttgaatctttacctacacattactcaggcattgcatttaaaatatatgagggttctaaaaatttttatccttgcgttgaaataaaggcttctcccgcaaaagtattacagggtcataatgtttttggtacaaccgatttagctttatgctctgaggctttattgcttaattttgctaattctttgccttgcctgtatgatttattggatgttggaatcgcctgatgcggtattttctccttacgcatctgtgcggtatttcacaccgcatatggtgcactctcagtacaatctgctctgatgccgcatagttaagccagccccgacacccgccaacactatggtgcactctcagtacaatctgctctgatgccgcatagttaagccagccccgacacccgccaacacccgctgacgcgccctgacgggcttgtctgctcccggcatccgcttacagacaagctgtgaccgtctccgggagctgcatgtgtcagaggttttcaccgtcatcaccgaaacgcgcgagacgaaagggcctcgtgatacgcctatttttataggttaatgtcatgataataatggtttcttagacgtcaggtggcacttttcggggaaatgtgcgcggaacccctatttgtttatttttctaaatacattcaaatatgtatccgctcatgagacaataaccctgataaatgcttcaataatattgaaaaaggaagagtatgagccatattcaacgggaaacgtcgaggccgcgattaaattccaacatggatgctgatttatatgggtataaatgggctcgcgataatgtcgggcaatcaggtgcgacaatctatcgcttgtatgggaagcccgatgcgccagagttgtttctgaaacatggcaaaggtagcgttgccaatgatgttacagatgagatggtcagactaaactggctgacggaatttatgccacttccgaccatcaagcattttatccgtactcctgatgatgcatggttactcaccactgcgatccccggaaaaacagcgttccaggtattagaagaatatcctgattcaggtgaaaatattgttgatgcgctggcagtgttcctgcgccggttgcactcgattcctgtttgtaattgtccttttaacagcgatcgcgtatttcgcctcgctcaggcgcaatcacgaatgaataacggtttggttgatgcgagtgattttgatgacgagcgtaatggctggcctgttgaacaagtctggaaagaaatgcataaacttttgccattctcaccggattcagtcgtcactcatggtgatttctcacttgataaccttatttttgacgaggggaaattaataggttgtattgatgttggacgagtcggaatcgcagaccgataccaggatcttgccatcctatggaactgcctcggtgagttttctccttcattacagaaacggctttttcaaaaatatggtattgataatcctgatatgaataaattgcagtttcatttgatgctcgatgagtttttctaactgtcagaccaagtttactcatatatactttagattgatttaaaacttcatttttaatttaaaaggatctaggtgaagatcctttttgataatctcatgaccaaaatcccttaacgtgagttttcgttccactgagcgtcagaccccgtagaaaagatcaaaggatcttcttgagatcctttttttctgcgcgtaatctgctgcttgcaaacaaaaaaaccaccgctaccagcggtggtttgtttgccggatcaagagctaccaactctttttccgaaggtaactggcttcagcagagcgcagataccaaatactgttcttctagtgtagccgtagttaggccaccacttcaagaactctgtagcaccgcctacatacctcgctctgctaatcctgttaccagtggctgctgccagtggcgataagtcgtgtcttaccgggttggactcaagacgatagttaccggataaggcgcagcggtcgggctgaacggggggttcgtgcacacagcccagcttggagcgaacgacctacaccgaactgagatacctacagcgtgagctatgagaaagcgccacgcttcccgaagggagaaaggcggacaggtatccggtaagcggcagggtcggaacaggagagcgcacgagggagcttccagggggaaacgcctggtatctttatagtcctgtcgggtttcgccacctctgacttgagcgtcgatttttgtgatgctcgtcaggggggcggagcctatggaaaaacgccagcaacgcggcctttttacggttcctggccttttgctggccttttgctcacatgttctttcctgcgttatcccctgattctgtggataaccgtattaccgcctttgagtgagctgataccgctcgccgcagccgaacgaccgagcgcagcgagtcagtgagcgaggaagcggaagagcgcccaatacgcaaaccgcctctccccgcgcgttggccgattcattaatgcagctggcgtaatagcgaagaggcccgcaccgatcgcccttcccaacagttgcgcagcctgaatggcgaatggcgattccgttgcaatggctggcggtaatattgttctggatattaccagcaaggccgatagtttgagttcttctactcaggcaagtgatgttattactaatcaaagaagtattgcgacaacggttaatttgcgtgatggacagactcttttactcggtggcctcactgattataaaaacacttctcaggattctggcgtaccgttcctgtctaaaatccctttaatcggcctcctgtttagctcccgctctgattctaacgaggaaagcacgttatacgtgctcgtcaaagcaaccatagtacgcgccctgtagcggcgcattaagcgcggcgggtgtggtggttacgcgcagcgtgaccgctacacttgccagcgccctagcgcccgctcctttcgctttcttcccttcctttctcgccacgttcgccggctttccccgtcaagctctaaatcgggggctccctttagggttccgatttagtgctttacggcacctcgaccccaaaaaacttgattagggtgatggttcacgtagtgggccatcgccctgatagacggtttttcgccctttgacgttggagtccacgttctttaatagtggactcttgttccaaactggaacaacactcaaccctatctcggtctattcttttgatttataagggattttgccgatttcggcctattggttaaaaaatgagctgatttaacaaaaatttaacgcgaattttaacaaaatattaacgcttacaatttaaatatttgcttatacaatcttcctgtttttggggcttttctgattatcaaccggggtacatatgattgacatgctagttttacgattaccgttcatcgcc

SEQ ID NO: 11 - DNA, 5998 bp, synthetic construct
  source 1..5998: mol_type = other DNA
ctgcgcgctcgctcgctcactgaggccgcccgggcaaagcccgggcgtcgggcgacctttggtcgcccggcctcagtgagcgagcgagcgcgcagagagggagtggaattcacgcgtggatctgaattcaattcacgcgtggtacctctggtcgttacataacttacggtaaatggcccgcctggctgaccgcccaacgacccccgcccattgacgtcaataatgacgtatgttcccatagtaacgccaatagggactttccattgacgtcaatgggtggagtatttacggtaaactgcccacttggcagtacatcaagtgtatcatatgccaagtacgccccctattgacgtcaatgacggtaaatggcccgcctggcattatgcccagtacatgaccttatgggactttcctacttggcagtacatctactcgaggccacgttctgcttcactctccccatctcccccccctccccacccccaattttgtatttatttattttttaattattttgtgcagcgatgggggcggggggggggggggggcgcgcgccaggcggggcggggcggggcgaggggcggggcggggcgaggcggagaggtgcggcggcagccaatcagagcggcgcgctccgaaagtttccttttatggcgaggcggcggcggcggcggccctataaaaagcgaagcgcgcggcgggcgggagcgggatcagccaccgcggtggcggcctagagtcgacgaggaactgaaaaaccagaaagttaactggtaagtttagtctttttgtcttttatttcaggtcccggatccggtggtggtgcaaatcaaagaactgctcctcagtggatgttgcctttacttctaggcctgtacggaagtgttacttctgctctaaaagctgcggaattgtacccgcggccgatggcaatgtcatcaggtggaagtggtggaggggtccctgaacaagaagacagcgtgttgtttaggcgcggcaccggacagagcgacgattctgatatctgggatgataccgcacttatcaaagcgtacgataaagctgttgcatcctttaagcacgctctcaagaacggagacatctgtgaaacgagcggcaagccaaagaccacccccaaaaggaagccagccaagaaaaataaatctcagaaaaaaaacaccgctgcaagccttcagcagtggaaggtcggtgataagtgcagcgccatttggagtgaggatggctgtatctatcctgccacaatcgcctctattgacttcaagcgcgaaacttgcgtggtagtgtataccggatatggcaatagagaggagcagaacctgtctgacctgctcagtccaatttgtgaggtcgcaaacaatattgagcagaacgcgcaggaaaatgaaaatgaatctcaggtcagcaccgatgagagcgagaattcaaggtctcccgggaataaatcagacaacatcaagcccaagtccgccccatggaattcctttttgccacctcctcctccgatgccaggacctagactgggaccaggtaaacctggtctgaagttcaatggacctcctccacctcctcctcctccaccaccacatcttctgagttgctggctgcccccctttccttctggtccccctataatccccccacctcctcccatatgccctgacagcctggatgacgccgatgccctgggaagtatgctgattagctggtacatgagcgggtaccacactggatactatatggggtttagacagaaccagaaggagggcagatgttctcactctctgaattgaagatctagaaagcttatcgataccgtcgactagagctcgctgatcagcctagtgaattctaccagtgccatataggtcaatgagggatgcaaacaccattgtcacactccaacttgggagtcctatgaagtgaattctaccagtgccataagactgatgtaaactagcaaacaccattgtcacactccacgactgtgccttctagttgccagccatctgttgtttgcccctcccccgtgccttccttgaccctggaaggtgccactcccactgtcctttcctaataaaatgaggaaattgcatcgcattgtctgagtaggtgtcattctattctggggggtggggtggggcaggacagcaagggggaggattgggaagacaatagcaggcatgctggggagagatcgatctgaggaacccctagtgatggagttggccactccctctctgcgcgctcgctcgctcactgaggccgggcgaccaaaggtcgcccgacgcccgggctttgcccgggcggcctcagtgagcgagcgagcgcgcagagagggagtggcccccccccccccccccccggcgattctcttgtttgctccagactctcaggcaatgacctgatagcctttgtagagacctctcaaaaatagctaccctctccggcatgaatttatcagctagaacggttgaatatcatattgatggtgatttgactgtctccggcctttctcacccgtttgaatctttacctacacattactcaggcattgcatttaaaatatatgagggttctaaaaatttttatccttgcgttgaaataaaggcttctcccgcaaaagtattacagggtcataatgtttttggtacaaccgatttagctttatgctctgaggctttattgcttaattttgctaattctttgccttgcctgtatgatttattggatgttggaatcgcctgatgcggtattttctccttacgcatctgtgcggtatttcacaccgcatatggtgcactctcagtacaatctgctctgatgccgcatagttaagccagccccgacacccgccaacactatggtgcactctcagtacaatctgctctgatgccgcatagttaagccagccccgacacccgccaacacccgctgacgcgccctgacgggcttgtctgctcccggcatccgcttacagacaagctgtgaccgtctccgggagctgcatgtgtcagaggttttcaccgtcatcaccgaaacgcgcgagacgaaagggcctcgtgatacgcctatttttataggttaatgtcatgataataatggtttcttagacgtcaggtggcacttttcggggaaatgtgcgcggaacccctatttgtttatttttctaaatacattcaaatatgtatccgctcatgagacaataaccctgataaatgcttcaataatattgaaaaaggaagagtatgagccatattcaacgggaaacgtcgaggccgcgattaaattccaacatggatgctgatttatatgggtataaatgggctcgcgataatgtcgggcaatcaggtgcgacaatctatcgcttgtatgggaagcccgatgcgccagagttgtttctgaaacatggcaaaggtagcgttgccaatgatgttacagatgagatggtcagactaaactggctgacggaatttatgccacttccgaccatcaagcattttatccgtactcctgatgatgcatggttactcaccactgcgatccccggaaaaacagcgttccaggtattagaagaatatcctgattcaggtgaaaatattgttgatgcgctggcagtgttcctgcgccggttgcactcgattcctgtttgtaattgtccttttaacagcgatcgcgtatttcgcctcgctcaggcgcaatcacgaatgaataacggtttggttgatgcgagtgattttgatgacgagcgtaatggctggcctgttgaacaagtctggaaagaaatgcataaacttttgccattctcaccggattcagtcgtcactcatggtgatttctcacttgataaccttatttttgacgaggggaaattaataggttgtattgatgttggacgagtcggaatcgcagaccgataccaggatcttgccatcctatggaactgcctcggtgagttttctccttcattacagaaacggctttttcaaaaatatggtattgataatcctgatatgaataaattgcagtttcatttgatgctcgatgagtttttctaactgtcagaccaagtttactcatatatactttagattgatttaaaacttcatttttaatttaaaaggatctaggtgaagatcctttttgataatctcatgaccaaaatcccttaacgtgagttttcgttccactgagcgtcagaccccgtagaaaagatcaaaggatcttcttgagatcctttttttctgcgcgtaatctgctgcttgcaaacaaaaaaaccaccgctaccagcggtggtttgtttgccggatcaagagctaccaactctttttccgaaggtaactggcttcagcagagcgcagataccaaatactgttcttctagtgtagccgtagttaggccaccacttcaagaactctgtagcaccgcctacatacctcgctctgctaatcctgttaccagtggctgctgccagtggcgataagtcgtgtcttaccgggttggactcaagacgatagttaccggataaggcgcagcggtcgggctgaacggggggttcgtgcacacagcccagcttggagcgaacgacctacaccgaactgagatacctacagcgtgagctatgagaaagcgccacgcttcccgaagggagaaaggcggacaggtatccggtaagcggcagggtcggaacaggagagcgcacgagggagcttccagggggaaacgcctggtatctttatagtcctgtcgggtttcgccacctctgacttgagcgtcgatttttgtgatgctcgtcaggggggcggagcctatggaaaaacgccagcaacgcggcctttttacggttcctggccttttgctggccttttgctcacatgttctttcctgcgttatcccctgattctgtggataaccgtattaccgcctttgagtgagctgataccgctcgccgcagccgaacgaccgagcgcagcgagtcagtgagcgaggaagcggaagagcgcccaatacgcaaaccgcctctccccgcgcgttggccgattcattaatgcagctggcgtaatagcgaagaggcccgcaccgatcgcccttcccaacagttgcgcagcctgaatggcgaatggcgattccgttgcaatggctggcggtaatattgttctggatattaccagcaaggccgatagtttgagttcttctactcaggcaagtgatgttattactaatcaaagaagtattgcgacaacggttaatttgcgtgatggacagactcttttactcggtggcctcactgattataaaaacacttctcaggattctggcgtaccgttcctgtctaaaatccctttaatcggcctcctgtttagctcccgctctgattctaacgaggaaagcacgttatacgtgctcgtcaaagcaaccatagtacgcgccctgtagcggcgcattaagcgcggcgggtgtggtggttacgcgcagcgtgaccgctacacttgccagcgccctagcgcccgctcctttcgctttcttcccttcctttctcgccacgttcgccggctttccccgtcaagctctaaatcgggggctccctttagggttccgatttagtgctttacggcacctcgaccccaaaaaacttgattagggtgatggttcacgtagtgggccatcgccctgatagacggtttttcgccctttgacgttggagtccacgttctttaatagtggactcttgttccaaactggaacaacactcaaccctatctcggtctattcttttgatttataagggattttgccgatttcggcctattggttaaaaaatgagctgatttaacaaaaatttaacgcgaattttaacaaaatattaacgcttacaatttaaatatttgcttatacaatcttcctgtttttggggcttttctgattatcaaccggggtacatatgattgacatgctagttttacgattaccgttcatcgcc

SEQ ID NO: 12 - DNA, 6004 bp, synthetic construct
  source 1..6004: mol_type = other DNA
ctgcgcgctcgctcgctcactgaggccgcccgggcaaagcccgggcgtcgggcgacctttggtcgcccggcctcagtgagcgagcgagcgcgcagagagggagtggaattcacgcgtggatctgaattcaattcacgcgtggtacctctggtcgttacataacttacggtaaatggcccgcctggctgaccgcccaacgacccccgcccattgacgtcaataatgacgtatgttcccatagtaacgccaatagggactttccattgacgtcaatgggtggagtatttacggtaaactgcccacttggcagtacatcaagtgtatcatatgccaagtacgccccctattgacgtcaatgacggtaaatggcccgcctggcattatgcccagtacatgaccttatgggactttcctacttggcagtacatctactcgaggccacgttctgcttcactctccccatctcccccccctccccacccccaattttgtatttatttattttttaattattttgtgcagcgatgggggcggggggggggggggggcgcgcgccaggcggggcggggcggggcgaggggcggggcggggcgaggcggagaggtgcggcggcagccaatcagagcggcgcgctccgaaagtttccttttatggcgaggcggcggcggcggcggccctataaaaagcgaagcgcgcggcgggcgggagcgggatcagccaccgcggtggcggcctagagtcgacgaggaactgaaaaaccagaaagttaactggtaagtttagtctttttgtcttttatttcaggtcccggatccggtggtggtgcaaatcaaagaactgctcctcagtggatgttgcctttacttctaggcctgtacggaagtgttacttctgctctaaaagctgcggaattgtacccgcggccggccaccatggctatgtctagtggtggatctggtggcggcgtgcccgagcaagaagatagcgtcctgttcagaagaggcaccggccagagcgacgacagcgacatctgggatgatacagccctgatcaaggcctacgacaaggccgtggccagctttaagcacgccctgaagaacggcgatatctgcgagacaagcggcaagcccaagaccacacctaagagaaagcccgccaagaagaacaagagccagaagaagaataccgccgccagcctgcagcagtggaaagtgggcgataagtgcagcgccatttggagcgaggacggctgtatctaccctgccacaatcgccagcatcgacttcaagcgggaaacctgcgtggtggtgtacacaggctacggcaacagagaggaacagaacctgagcgacctgctgagcccaatttgcgaggtggccaacaacatcgagcagaacgcccaagagaacgagaacgagtcccaggtgtccaccgacgagagcgagaatagcagaagccccggcaacaagagcgacaacatcaagcctaagagcgccccttggaacagcttcctgcctcctcctccaccaatgcctggacctagactcggacctggaaagcccggcctgaagttcaatggacctccaccaccgccaccacctccgcctccacatcttctgtcttgttggctgcctccatttcctagcggccctccaatcatcccgccacctccacctatctgccccgacagtctggatgatgctgatgccctgggctccatgctgatctcttggtacatgagcggctaccacaccggctactacatgggcttcagacagaaccagaaagagggccgttgcagccacagcctgaactgaagatctagaaagcttatcgataccgtcgactagagctcgctgatcagcctagtgaattctaccagtgccatataggtcaatgagggatgcaaacaccattgtcacactccaacttgggagtcctatgaagtgaattctaccagtgccataagactgatgtaaactagcaaacaccattgtcacactccacgactgtgccttctagttgccagccatctgttgtttgcccctcccccgtgccttccttgaccctggaaggtgccactcccactgtcctttcctaataaaatgaggaaattgcatcgcattgtctgagtaggtgtcattctattctggggggtggggtggggcaggacagcaagggggaggattgggaagacaatagcaggcatgctggggagagatcgatctgaggaacccctagtgatggagttggccactccctctctgcgcgctcgctcgctcactgaggccgggcgaccaaaggtcgcccgacgcccgggctttgcccgggcggcctcagtgagcgagcgagcgcgcagagagggagtggcccccccccccccccccccggcgattctcttgtttgctccagactctcaggcaatgacctgatagcctttgtagagacctctcaaaaatagctaccctctccggcatgaatttatcagctagaacggttgaatatcatattgatggtgatttgactgtctccggcctttctcacccgtttgaatctttacctacacattactcaggcattgcatttaaaatatatgagggttctaaaaatttttatccttgcgttgaaataaaggcttctcccgcaaaagtattacagggtcataatgtttttggtacaaccgatttagctttatgctctgaggctttattgcttaattttgctaattctttgccttgcctgtatgatttattggatgttggaatcgcctgatgcggtattttctccttacgcatctgtgcggtatttcacaccgcatatggtgcactctcagtacaatctgctctgatgccgcatagttaagccagccccgacacccgccaacactatggtgcactctcagtacaatctgctctgatgccgcatagttaagccagccccgacacccgccaacacccgctgacgcgccctgacgggcttgtctgctcccggcatccgcttacagacaagctgtgaccgtctccgggagctgcatgtgtcagaggttttcaccgtcatcaccgaaacgcgcgagacgaaagggcctcgtgatacgcctatttttataggttaatgtcatgataataatggtttcttagacgtcaggtggcacttttcggggaaatgtgcgcggaacccctatttgtttatttttctaaatacattcaaatatgtatccgctcatgagacaataaccctgataaatgcttcaataatattgaaaaaggaagagtatgagccatattcaacgggaaacgtcgaggccgcgattaaattccaacatggatgctgatttatatgggtataaatgggctcgcgataatgtcgggcaatcaggtgcgacaatctatcgcttgtatgggaagcccgatgcgccagagttgtttctgaaacatggcaaaggtagcgttgccaatgatgttacagatgagatggtcagactaaactggctgacggaatttatgccacttccgaccatcaagcattttatccgtactcctgatgatgcatggttactcaccactgcgatccccggaaaaacagcgttccaggtattagaagaatatcctgattcaggtgaaaatattgttgatgcgctggcagtgttcctgcgccggttgcactcgattcctgtttgtaattgtccttttaacagcgatcgcgtatttcgcctcgctcaggcgcaatcacgaatgaataacggtttggttgatgcgagtgattttgatgacgagcgtaatggctggcctgttgaacaagtctggaaagaaatgcataaacttttgccattctcaccggattcagtcgtcactcatggtgatttctcacttgataaccttatttttgacgaggggaaattaataggttgtattgatgttggacgagtcggaatcgcagaccgataccaggatcttgccatcctatggaactgcctcggtgagttttctccttcattacagaaacggctttttcaaaaatatggtattgataatcctgatatgaataaattgcagtttcatttgatgctcgatgagtttttctaactgtcagaccaagtttactcatatatactttagattgatttaaaacttcatttttaatttaaaaggatctaggtgaagatcctttttgataatctcatgaccaaaatcccttaacgtgagttttcgttccactgagcgtcagaccccgtagaaaagatcaaaggatcttcttgagatcctttttttctgcgcgtaatctgctgcttgcaaacaaaaaaaccaccgctaccagcggtggtttgtttgccggatcaagagctaccaactctttttccgaaggtaactggcttcagcagagcgcagataccaaatactgttcttctagtgtagccgtagttaggccaccacttcaagaactctgtagcaccgcctacatacctcgctctgctaatcctgttaccagtggctgctgccagtggcgataagtcgtgtcttaccgggttggactcaagacgatagttaccggataaggcgcagcggtcgggctgaacggggggttcgtgcacacagcccagcttggagcgaacgacctacaccgaactgagatacctacagcgtgagctatgagaaagcgccacgcttcccgaagggagaaaggcggacaggtatccggtaagcggcagggtcggaacaggagagcgcacgagggagcttccagggggaaacgcctggtatctttatagtcctgtcgggtttcgccacctctgacttgagcgtcgatttttgtgatgctcgtcaggggggcggagcctatggaaaaacgccagcaacgcggcctttttacggttcctggccttttgctggccttttgctcacatgttctttcctgcgttatcccctgattctgtggataaccgtattaccgcctttgagtgagctgataccgctcgccgcagccgaacgaccgagcgcagcgagtcagtgagcgaggaagcggaagagcgcccaatacgcaaaccgcctctccccgcgcgttggccgattcattaatgcagctggcgtaatagcgaagaggcccgcaccgatcgcccttcccaacagttgcgcagcctgaatggcgaatggcgattccgttgcaatggctggcggtaatattgttctggatattaccagcaaggccgatagtttgagttcttctactcaggcaagtgatgttattactaatcaaagaagtattgcgacaacggttaatttgcgtgatggacagactcttttactcggtggcctcactgattataaaaacacttctcaggattctggcgtaccgttcctgtctaaaatccctttaatcggcctcctgtttagctcccgctctgattctaacgaggaaagcacgttatacgtgctcgtcaaagcaaccatagtacgcgccctgtagcggcgcattaagcgcggcgggtgtggtggttacgcgcagcgtgaccgctacacttgccagcgccctagcgcccgctcctttcgctttcttcccttcctttctcgccacgttcgccggctttccccgtcaagctctaaatcgggggctccctttagggttccgatttagtgctttacggcacctcgaccccaaaaaacttgattagggtgatggttcacgtagtgggccatcgccctgatagacggtttttcgccctttgacgttggagtccacgttctttaatagtggactcttgttccaaactggaacaacactcaaccctatctcggtctattcttttgatttataagggattttgccgatttcggcctattggttaaaaaatgagctgatttaacaaaaatttaacgcgaattttaacaaaatattaacgcttacaatttaaatatttgcttatacaatcttcctgtttttggggcttttctgattatcaaccggggtacatatgattgacatgctagttttacgattaccgttcatcgcc

SEQ ID NO: 13 - DNA, 5859 bp, synthetic construct
  source 1..5859: mol_type = other DNA
ctgcgcgctcgctcgctcactgaggccgcccgggcaaagcccgggcgtcgggcgacctttggtcgcccggcctcagtgagcgagcgagcgcgcagagagggagtggaattcacgcgtggatctgaattcaattcacgcgtggtacctctggtcgttacataacttacggtaaatggcccgcctggctgaccgcccaacgacccccgcccattgacgtcaataatgacgtatgttcccatagtaacgccaatagggactttccattgacgtcaatgggtggagtatttacggtaaactgcccacttggcagtacatcaagtgtatcatatgccaagtacgccccctattgacgtcaatgacggtaaatggcccgcctggcattatgcccagtacatgaccttatgggactttcctacttggcagtacatctactcgaggccacgttctgcttcactctccccatctcccccccctccccacccccaattttgtatttatttattttttaattattttgtgcagcgatgggggcggggggggggggggggcgcgcgccaggcggggcggggcggggcgaggggcggggcggggcgaggcggagaggtgcggcggcagccaatcagagcggcgcgctccgaaagtttccttttatggcgaggcggcggcggcggcggccctataaaaagcgaagcgcgcggcgggcgggagcgggatcagccaccgcggtggcggcctagagtcgacgaggaactgaaaaaccagaaagttaactggtaagtttagtctttttgtcttttatttcaggtcccggatccggtggtggtgcaaatcaaagaactgctcctcagtggatgttgcctttacttctaggcctgtacggaagtgttacttctgctctaaaagctgcggaattgtacccgcggccgatggcaatgtcatcaggtggaagtggtggaggggtccctgaacaagaagacagcgtgttgtttaggcgcggcaccggacagagcgacgattctgatatctgggatgataccgcacttatcaaagcgtacgataaagctgttgcatcctttaagcacgctctcaagaacggagacatctgtgaaacgagcggcaagccaaagaccacccccaaaaggaagccagccaagaaaaataaatctcagaaaaaaaacaccgctgcaagccttcagcagtggaaggtcggtgataagtgcagcgccatttggagtgaggatggctgtatctatcctgccacaatcgcctctattgacttcaagcgcgaaacttgcgtggtagtgtataccggatatggcaatagagaggagcagaacctgtctgacctgctcagtccaatttgtgaggtcgcaaacaatattgagcagaacgcgcaggaaaatgaaaatgaatctcaggtcagcaccgatgagagcgagaattcaaggtctcccgggaataaatcagacaacatcaagcccaagtccgccccatggaattcctttttgccacctcctcctccgatgccaggacctagactgggaccaggtaaacctggtctgaagttcaatggacctcctccacctcctcctcctccaccaccacatcttctgagttgctggctgcccccctttccttctggtccccctataatccccccacctcctcccatatgccctgacagcctggatgacgccgatgccctgggaagtatgctgattagctggtacatgagcgggtaccacactggatactatatggggtttagacagaaccagaaggagggcagatgttctcactctctgaattgaagatctagaaagcttatcgataccgtcgactagagctcgctgatcagcctcgactgtgccttctagttgccagccatctgttgtttgcccctcccccgtgccttccttgaccctggaaggtgccactcccactgtcctttcctaataaaatgaggaaattgcatcgcattgtctgagtaggtgtcattctattctggggggtggggtggggcaggacagcaagggggaggattgggaagacaatagcaggcatgctggggagagatcgatctgaggaacccctagtgatggagttggccactccctctctgcgcgctcgctcgctcactgaggccgggcgaccaaaggtcgcccgacgcccgggctttgcccgggcggcctcagtgagcgagcgagcgcgcagagagggagtggcccccccccccccccccccggcgattctcttgtttgctccagactctcaggcaatgacctgatagcctttgtagagacctctcaaaaatagctaccctctccggcatgaatttatcagctagaacggttgaatatcatattgatggtgatttgactgtctccggcctttctcacccgtttgaatctttacctacacattactcaggcattgcatttaaaatatatgagggttctaaaaatttttatccttgcgttgaaataaaggcttctcccgcaaaagtattacagggtcataatgtttttggtacaaccgatttagctttatgctctgaggctttattgcttaattttgctaattctttgccttgcctgtatgatttattggatgttggaatcgcctgatgcggtattttctccttacgcatctgtgcggtatttcacaccgcatatggtgcactctcagtacaatctgctctgatgccgcatagttaagccagccccgacacccgccaacactatggtgcactctcagtacaatctgctctgatgccgcatagttaagccagccccgacacccgccaacacccgctgacgcgccctgacgggcttgtctgctcccggcatccgcttacagacaagctgtgaccgtctccgggagctgcatgtgtcagaggttttcaccgtcatcaccgaaacgcgcgagacgaaagggcctcgtgatacgcctatttttataggttaatgtcatgataataatggtttcttagacgtcaggtggcacttttcggggaaatgtgcgcggaacccctatttgtttatttttctaaatacattcaaatatgtatccgctcatgagacaataaccctgataaatgcttcaataatattgaaaaaggaagagtatgagccatattcaacgggaaacgtcgaggccgcgattaaattccaacatggatgctgatttatatgggtataaatgggctcgcgataatgtcgggcaatcaggtgcgacaatctatcgcttgtatgggaagcccgatgcgccagagttgtttctgaaacatggcaaaggtagcgttgccaatgatgttacagatgagatggtcagactaaactggctgacggaatttatgccacttccgaccatcaagcattttatccgtactcctgatgatgcatggttactcaccactgcgatccccggaaaaacagcgttccaggtattagaagaatatcctgattcaggtgaaaatattgttgatgcgctggcagtgttcctgcgccggttgcactcgattcctgtttgtaattgtccttttaacagcgatcgcgtatttcgcctcgctcaggcgcaatcacgaatgaataacggtttggttgatgcgagtgattttgatgacgagcgtaatggctggcctgttgaacaagtctggaaagaaatgcataaacttttgccattctcaccggattcagtcgtcactcatggtgatttctcacttgataaccttatttttgacgaggggaaattaataggttgtattgatgttggacgagtcggaatcgcagaccgataccaggatcttgccatcctatggaactgcctcggtgagttttctccttcattacagaaacggctttttcaaaaatatggtattgataatcctgatatgaataaattgcagtttcatttgatgctcgatgagtttttctaactgtcagaccaagtttactcatatatactttagattgatttaaaacttcatttttaatttaaaaggatctaggtgaagatcctttttgataatctcatgaccaaaatcccttaacgtgagttttcgttccactgagcgtcagaccccgtagaaaagatcaaaggatcttcttgagatcctttttttctgcgcgtaatctgctgcttgcaaacaaaaaaaccaccgctaccagcggtggtttgtttgccggatcaagagctaccaactctttttccgaaggtaactggcttcagcagagcgcagataccaaatactgttcttctagtgtagccgtagttaggccaccacttcaagaactctgtagcaccgcctacatacctcgctctgctaatcctgttaccagtggctgctgccagtggcgataagtcgtgtcttaccgggttggactcaagacgatagttaccggataaggcgcagcggtcgggctgaacggggggttcgtgcacacagcccagcttggagcgaacgacctacaccgaactgagatacctacagcgtgagctatgagaaagcgccacgcttcccgaagggagaaaggcggacaggtatccggtaagcggcagggtcggaacaggagagcgcacgagggagcttccagggggaaacgcctggtatctttatagtcctgtcgggtttcgccacctctgacttgagcgtcgatttttgtgatgctcgtcaggggggcggagcctatggaaaaacgccagcaacgcggcctttttacggttcctggccttttgctggccttttgctcacatgttctttcctgcgttatcccctgattctgtggataaccgtattaccgcctttgagtgagctgataccgctcgccgcagccgaacgaccgagcgcagcgagtcagtgagcgaggaagcggaagagcgcccaatacgcaaaccgcctctccccgcgcgttggccgattcattaatgcagctggcgtaatagcgaagaggcccgcaccgatcgcccttcccaacagttgcgcagcctgaatggcgaatggcgattccgttgcaatggctggcggtaatattgttctggatattaccagcaaggccgatagtttgagttcttctactcaggcaagtgatgttattactaatcaaagaagtattgcgacaacggttaatttgcgtgatggacagactcttttactcggtggcctcactgattataaaaacacttctcaggattctggcgtaccgttcctgtctaaaatccctttaatcggcctcctgtttagctcccgctctgattctaacgaggaaagcacgttatacgtgctcgtcaaagcaaccatagtacgcgccctgtagcggcgcattaagcgcggcgggtgtggtggttacgcgcagcgtgaccgctacacttgccagcgccctagcgcccgctcctttcgctttcttcccttcctttctcgccacgttcgccggctttccccgtcaagctctaaatcgggggctccctttagggttccgatttagtgctttacggcacctcgaccccaaaaaacttgattagggtgatggttcacgtagtgggccatcgccctgatagacggtttttcgccctttgacgttggagtccacgttctttaatagtggactcttgttccaaactggaacaacactcaaccctatctcggtctattcttttgatttataagggattttgccgatttcggcctattggttaaaaaatgagctgatttaacaaaaatttaacgcgaattttaacaaaatattaacgcttacaatttaaatatttgcttatacaatcttcctgtttttggggcttttctgattatcaaccggggtacatatgattgacatgctagttttacgattaccgttcatcgcc

SEQ ID NO: 14 - DNA, 5865 bp, synthetic construct
  source 1..5865: mol_type = other DNA
ctgcgcgctcgctcgctcactgaggccgcccgggcaaagcccgggcgtcgggcgacctttggtcgcccggcctcagtgagcgagcgagcgcgcagagagggagtggaattcacgcgtggatctgaattcaattcacgcgtggtacctctggtcgttacataacttacggtaaatggcccgcctggctgaccgcccaacgacccccgcccattgacgtcaataatgacgtatgttcccatagtaacgccaatagggactttccattgacgtcaatgggtggagtatttacggtaaactgcccacttggcagtacatcaagtgtatcatatgccaagtacgccccctattgacgtcaatgacggtaaatggcccgcctggcattatgcccagtacatgaccttatgggactttcctacttggcagtacatctactcgaggccacgttctgcttcactctccccatctcccccccctccccacccccaattttgtatttatttattttttaattattttgtgcagcgatgggggcggggggggggggggggcgcgcgccaggcggggcggggcggggcgaggggcggggcggggcgaggcggagaggtgcggcggcagccaatcagagcggcgcgctccgaaagtttccttttatggcgaggcggcggcggcggcggccctataaaaagcgaagcgcgcggcgggcgggagcgggatcagccaccgcggtggcggcctagagtcgacgaggaactgaaaaaccagaaagttaactggtaagtttagtctttttgtcttttatttcaggtcccggatccggtggtggtgcaaatcaaagaactgctcctcagtggatgttgcctttacttctaggcctgtacggaagtgttacttctgctctaaaagctgcggaattgtacccgcggccggccaccatggctatgtctagtggtggatctggtggcggcgtgcccgagcaagaagatagcgtcctgttcagaagaggcaccggccagagcgacgacagcgacatctgggatgatacagccctgatcaaggcctacgacaaggccgtggccagctttaagcacgccctgaagaacggcgatatctgcgagacaagcggcaagcccaagaccacacctaagagaaagcccgccaagaagaacaagagccagaagaagaataccgccgccagcctgcagcagtggaaagtgggcgataagtgcagcgccatttggagcgaggacggctgtatctaccctgccacaatcgccagcatcgacttcaagcgggaaacctgcgtggtggtgtacacaggctacggcaacagagaggaacagaacctgagcgacctgctgagcccaatttgcgaggtggccaacaacatcgagcagaacgcccaagagaacgagaacgagtcccaggtgtccaccgacgagagcgagaatagcagaagccccggcaacaagagcgacaacatcaagcctaagagcgccccttggaacagcttcctgcctcctcctccaccaatgcctggacctagactcggacctggaaagcccggcctgaagttcaatggacctccaccaccgccaccacctccgcctccacatcttctgtcttgttggctgcctccatttcctagcggccctccaatcatcccgccacctccacctatctgccccgacagtctggatgatgctgatgccctgggctccatgctgatctcttggtacatgagcggctaccacaccggctactacatgggcttcagacagaaccagaaagagggccgttgcagccacagcctgaactgaagatctagaaagcttatcgataccgtcgactagagctcgctgatcagcctcgactgtgccttctagttgccagccatctgttgtttgcccctcccccgtgccttccttgaccctggaaggtgccactcccactgtcctttcctaataaaatgaggaaattgcatcgcattgtctgagtaggtgtcattctattctggggggtggggtggggcaggacagcaagggggaggattgggaagacaatagcaggcatgctggggagagatcgatctgaggaacccctagtgatggagttggccactccctctctgcgcgctcgctcgctcactgaggccgggcgaccaaaggtcgcccgacgcccgggctttgcccgggcggcctcagtgagcgagcgagcgcgcagagagggagtggcccccccccccccccccccggcgattctcttgtttgctccagactctcaggcaatgacctgatagcctttgtagagacctctcaaaaatagctaccctctccggcatgaatttatcagctagaacggttgaatatcatattgatggtgatttgactgtctccggcctttctcacccgtttgaatctttacctacacattactcaggcattgcatttaaaatatatgagggttctaaaaatttttatccttgcgttgaaataaaggcttctcccgcaaaagtattacagggtcataatgtttttggtacaaccgatttagctttatgctctgaggctttattgcttaattttgctaattctttgccttgcctgtatgatttattggatgttggaatcgcctgatgcggtattttctccttacgcatctgtgcggtatttcacaccgcatatggtgcactctcagtacaatctgctctgatgccgcatagttaagccagccccgacacccgccaacactatggtgcactctcagtacaatctgctctgatgccgcatagttaagccagccccgacacccgccaacacccgctgacgcgccctgacgggcttgtctgctcccggcatccgcttacagacaagctgtgaccgtctccgggagctgcatgtgtcagaggttttcaccgtcatcaccgaaacgcgcgagacgaaagggcctcgtgatacgcctatttttataggttaatgtcatgataataatggtttcttagacgtcaggtggcacttttcggggaaatgtgcgcggaacccctatttgtttatttttctaaatacattcaaatatgtatccgctcatgagacaataaccctgataaatgcttcaataatattgaaaaaggaagagtatgagccatattcaacgggaaacgtcgaggccgcgattaaattccaacatggatgctgatttatatgggtataaatgggctcgcgataatgtcgggcaatcaggtgcgacaatctatcgcttgtatgggaagcccgatgcgccagagttgtttctgaaacatggcaaaggtagcgttgccaatgatgttacagatgagatggtcagactaaactggctgacggaatttatgccacttccgaccatcaagcattttatccgtactcctgatgatgcatggttactcaccactgcgatccccggaaaaacagcgttccaggtattagaagaatatcctgattcaggtgaaaatattgttgatgcgctggcagtgttcctgcgccggttgcactcgattcctgtttgtaattgtccttttaacagcgatcgcgtatttcgcctcgctcaggcgcaatcacgaatgaataacggtttggttgatgcgagtgattttgatgacgagcgtaatggctggcctgttgaacaagtctggaaagaaatgcataaacttttgccattctcaccggattcagtcgtcactcatggtgatttctcacttgataaccttatttttgacgaggggaaattaataggttgtattgatgttggacgagtcggaatcgcagaccgataccaggatcttgccatcctatggaactgcctcggtgagttttctccttcattacagaaacggctttttcaaaaatatggtattgataatcctgatatgaataaattgcagtttcatttgatgctcgatgagtttttctaactgtcagaccaagtttactcatatatactttagattgatttaaaacttcatttttaatttaaaaggatctaggtgaagatcctttttgataatctcatgaccaaaatcccttaacgtgagttttcgttccactgagcgtcagaccccgtagaaaagatcaaaggatcttcttgagatcctttttttctgcgcgtaatctgctgcttgcaaacaaaaaaaccaccgctaccagcggtggtttgtttgccggatcaagagctaccaactctttttccgaaggtaactggcttcagcagagcgcagataccaaatactgttcttctagtgtagccgtagttaggccaccacttcaagaactctgtagcaccgcctacatacctcgctctgctaatcctgttaccagtggctgctgccagtggcgataagtcgtgtcttaccgggttggactcaagacgatagttaccggataaggcgcagcggtcgggctgaacggggggttcgtgcacacagcccagcttggagcgaacgacctacaccgaactgagatacctacagcgtgagctatgagaaagcgccacgcttcccgaagggagaaaggcggacaggtatccggtaagcggcagggtcggaacaggagagcgcacgagggagcttccagggggaaacgcctggtatctttatagtcctgtcgggtttcgccacctctgacttgagcgtcgatttttgtgatgctcgtcaggggggcggagcctatggaaaaacgccagcaacgcggcctttttacggttcctggccttttgctggccttttgctcacatgttctttcctgcgttatcccctgattctgtggataaccgtattaccgcctttgagtgagctgataccgctcgccgcagccgaacgaccgagcgcagcgagtcagtgagcgaggaagcggaagagcgcccaatacgcaaaccgcctctccccgcgcgttggccgattcattaatgcagctggcgtaatagcgaagaggcccgcaccgatcgcccttcccaacagttgcgcagcctgaatggcgaatggcgattccgttgcaatggctggcggtaatattgttctggatattaccagcaaggccgatagtttgagttcttctactcaggcaagtgatgttattactaatcaaagaagtattgcgacaacggttaatttgcgtgatggacagactcttttactcggtggcctcactgattataaaaacacttctcaggattctggcgtaccgttcctgtctaaaatccctttaatcggcctcctgtttagctcccgctctgattctaacgaggaaagcacgttatacgtgctcgtcaaagcaaccatagtacgcgccctgtagcggcgcattaagcgcggcgggtgtggtggttacgcgcagcgtgaccgctacacttgccagcgccctagcgcccgctcctttcgctttcttcccttcctttctcgccacgttcgccggctttccccgtcaagctctaaatcgggggctccctttagggttccgatttagtgctttacggcacctcgaccccaaaaaacttgattagggtgatggttcacgtagtgggccatcgccctgatagacggtttttcgccctttgacgttggagtccacgttctttaatagtggactcttgttccaaactggaacaacactcaaccctatctcggtctattcttttgatttataagggattttgccgatttcggcctattggttaaaaaatgagctgatttaacaaaaatttaacgcgaattttaacaaaatattaacgcttacaatttaaatatttgcttatacaatcttcctgtttttggggcttttctgattatcaaccggggtacatatgattgacatgctagttttacgattaccgttcatcgcc

SEQ ID NO: 15 - DNA, 37 bp, synthetic construct
  source 1..37: mol_type = other DNA
gatcagcctcgactgtgccttctagttgccagccatc

SEQ ID NO: 16 - DNA, 37 bp, synthetic construct
  source 1..37: mol_type = other DNA
gcacagtcgaggctgatcagcgagctctagtcgacgg

SEQ ID NO: 17 - DNA, 22 bp, synthetic construct
  source 1..22: mol_type = other DNA
ttttctccctcttcagagtgat

SEQ ID NO: 18 - DNA, 21 bp, synthetic construct
  source 1..21: mol_type = other DNA
ctgtttcaagggagttgtggc

SEQ ID NO: 19 - DNA, 19 bp, synthetic construct
  source 1..19: mol_type = other DNA
ctccgggatattgggattg

SEQ ID NO: 20 - DNA, 19 bp, synthetic construct
  source 1..19: mol_type = other DNA
ggtaacgccagggttttcc

SEQ ID NO: 21 - DNA, 22 bp, synthetic construct
  source 1..22: mol_type = other DNA
agtgaattctaccagtgccata

SEQ ID NO: 22 - DNA, 22 bp, synthetic construct
  source 1..22: mol_type = other DNA
caaacaccattgtcacactcca

SEQ ID NO: 23 - DNA, 53 bp, synthetic construct
  source 1..53: mol_type = other DNA
aactatacaacctactacctcagttttataaagagtttgccttataaatttac

SEQ ID NO: 24 - DNA, 49 bp, synthetic construct
  source 1..49: mol_type = other DNA
tgaggtagtaggttgtatagttccggttcagacaggtttactgaaatgg

SEQ ID NO: 25 - DNA, 53 bp, synthetic construct
  source 1..53: mol_type = other DNA
cacaagatcggatctacgggttgttttataaagagtttgccttataaatttac

SEQ ID NO: 26 - DNA, 49 bp, synthetic construct
  source 1..49: mol_type = other DNA
aacccgtagatccgatcttgtgccggttcagacaggtttactgaaatgg

SEQ ID NO: 27 - DNA, 53 bp, synthetic construct
  source 1..53: mol_type = other DNA
cacaagttcggatctacgggttgttttataaagagtttgccttataaatttac

SEQ ID NO: 28 - DNA, 49 bp, synthetic construct
  source 1..49: mol_type = other DNA
aacccgtagatccgaacttgtgccggttcagacaggtttactgaaatgg

SEQ ID NO: 29 - DNA, 54 bp, synthetic construct
  source 1..54: mol_type = other DNA
acaaggatgaatctttgttactggttttataaagagtttgccttataaatttac

SEQ ID NO: 30 - DNA, 50 bp, synthetic construct
  source 1..50: mol_type = other DNA
cagtaacaaagattcatccttgtccggttcagacaggtttactgaaatgg

SEQ ID NO: 31 - DNA, 53 bp, synthetic construct
  source 1..53: mol_type = other DNA
gaggctcagaatggctcaggaggttttataaagagtttgccttataaatttac

SEQ ID NO: 32 - DNA, 49 bp, synthetic construct
  source 1..49: mol_type = other DNA
ctcctgagccattctgagcctcccggttcagacaggtttactgaaatgg

SEQ ID NO: 33 - DNA, 4285 bp, synthetic construct
  source 1..4285: mol_type = other DNA
tcgcgcgtttcggtgatgacggtgaaaacctctgacacatgcagctcccggacgtcattgtcgatgctagcctgcgcgctcgctcgctcactgaggccgcccgggcaaagcccgggcgtcgggcgacctttggtcgcccggcctcagtgagcgagcgagcgcgcagagagggagtggataggcgccaagagcctagacttccttaagcgccagagtccacaagggcccagttaatcctcaacattcaaatgctgcccacaaaaccagcccctctgtgccctagccgcctcttttttccaagtgacagtagaactccaccaatccgcagctgaatggggtccgcctcttttccctgcctaaacagacaggaactcctgccaattgagggcgtcaccgctaaggctccgccccagcctgggctccacaaccaatgaagggtaatctcgacaaagagcaaggggtggggcgcgggcgcgcaggtgcagcagcacacaggctggtcgggagggcggggcgcgacgtctgccgtgcggggtcccggcatcggttgcgcgcgcgctccctcctctcggagagagggctgtggtaaaacccgtccggaaaccatggccgccgccgccgccgccgcgccgagcggaggaggaggaggaggcgaggaggagagactggaagaaaagtcagaagaccaggacctccagggcctcaaggacaaacccctcaagtttaaaaaggtgaagaaagataagaaagaagagaaagagggcaagcatgagcccgtgcagccatcagcccaccactctgctgagcccgcagaggcaggcaaagcagagacatcagaagggtcaggctccgccccggctgtgccggaagcttctgcctcccccaaacagcggcgctccatcatccgtgaccggggacccatgtatgatgaccccaccctgcctgaaggctggacacggaagcttaagcaaaggaaatctggccgctctgctgggaagtatgatgtgtatttgatcaatccccagggaaaagcctttcgctctaaagtggagttgattgcgtacttcgaaaaggtaggcgacacatccctggaccctaatgattttgacttcacggtaactgggagagggagcccctcccggcgagagcagaaaccacctaagaagcccaaatctcccaaagctccaggaactggcagaggccggggacgccccaaagggagcggcaccacgagacccaaggcggccacgtcagagggtgtgcaggtgaaaagggtcctggagaaaagtcctgggaagctccttgtcaagatgccttttcaaacttcgccagggggcaaggctgaggggggtggggccaccacatccacccaggtcatggtgatcaaacgccccggcaggaagcgaaaagctgaggccgaccctcaggccattcccaagaaacggggccgaaagccggggagtgtggtggcagccgctgccgccgaggccaaaaagaaagccgtgaaggagtcttctatccgatctgtgcaggagaccgtactccccatcaagaagcgcaagacccgggagacggtcagcatcgaggtcaaggaagtggtgaagcccctgctggtgtccaccctcggtgagaagagcgggaaaggactgaagacctgtaagagccctgggcggaaaagcaaggagagcagccccaaggggcgcagcagcagcgcctcctcaccccccaagaaggagcaccaccaccatcaccaccactcagagtccccaaaggcccccgtgccactgctcccacccctgcccccacctccacctgagcccgagagctccgaggaccccaccagcccccctgagccccaggacttgagcagcagcgtctgcaaagaggagaagatgcccagaggaggctcactggagagcgacggctgccccaaggagccagctaagactcagcccgcggttgccaccgccgccacggccgcagaaaagtacaaacaccgaggggagggagagcgcaaagacattgtttcatcctccatgccaaggccaaacagagaggagcctgtggacagccggacgcccgtgaccgagagagttagcgggagctccggcagttctggagaacaaaaactcatctcagaagaggatctgtgaacaagaataaaggcagctgttgtctcttctccttatgggtagggctctgacaaagcttcccatatcaccaggactgttaatatatttaaaaacaaaaggcaatttattaaggaaatttgtaccatttcagtaaacctgtctgaaccggaactatacaacctactacctcagttttataaagagtttgccttataaatttacataaaaatgtccgtttgtgtcttttgttgaggaacccctagtgatggagttggccactccctctctgcgcgctcgctcgctcactgaggccgggcgaccaaaggtcgcccgacgcccgggctttgcccgggcggcctcagtgagcgagcgagcgcgcagagagggagtggccatcattgtcacatgtgagcaaaaggccagcaaaaggccaggaaccgtaaaaaggccgcgttgctggcgtttttccataggctccgcccccctgacgagcatcacaaaaatcgacgctcaagtcagaggtggcgaaacccgacaggactataaagataccaggcgtttccccctggaagctccctcgtgcgctctcctgttccgaccctgccgcttaccggatacctgtccgcctttctcccttcgggaagcgtggcgctttctcatagctcacgctgtaggtatctcagttcggtgtaggtcgttcgctccaagctgggctgtgtgcacgaaccccccgttcagcccgaccgctgcgccttatccggtaactatcgtcttgagtccaacccggtaagacacgacttatcgccactggcagcagccactggtaacaggattagcagagcgaggtatgtaggcggtgctacagagttcttgaagtggtggcctaactacggctacactagaagaacagtatttggtatctgcgctctgctgaagccagttaccttcggaaaaagagttggtagctcttgatccggcaaacaaaccaccgctggtagcggtggtttttttgtttgcaagcagcagattacgcgcagaaaaaaaggatctcaagaagatcctttgatcttttctacggggtctgacgctcagtggaacgaaaactcacgttaagggattttggtcatgagattatcaaaaaggatcttcacctagatccttttaaattaaaaatgaagttttaaatcaagcccaatctgaataatgttacaaccaattaaccaattctgattagaaaaactcatcgagcatcaaatgaaactgcaatttattcatatcaggattatcaataccatatttttgaaaaagccgtttctgtaatgaaggagaaaactcaccgaggcagttccataggatggcaagatcctggtatcggtctgcgattccgactcgtccaacatcaatacaacctattaatttcccctcgtcaaaaataaggttatcaagtgagaaatcaccatgagtgacgactgaatccggtgagaatggcaaaagtttatgcatttctttccagacttgttcaacaggccagccattacgctcgtcatcaaaatcactcgcatcaaccaaaccgttattcattcgtgattgcgcctgagcgagacgaaatacgcgatcgctgttaaaaggacaattacaaacaggaatcgaatgcaaccggcgcaggaacactgccagcgcatcaacaatattttcacctgaatcaggatattcttctaatacctggaatgctgtttttccggggatcgcagtggtgagtaaccatgcatcatcaggagtacggataaaatgcttgatggtcggaagaggcataaattccgtcagccagtttagtctgaccatctcatctgtaacatcattggcaacgctacctttgccatgtttcagaaacaactctggcgcatcgggcttcccatacaagcgatagattgtcgcacctgattgcccgacattatcgcgagcccatttatacccatataaatcagcatccatgttggaatttaatcgcggcctcgacgtttcccgttgaatatggctcataacaccccttgtattactgtttatgtaagcagacagttttattgttcatgatgatatatttttatcttgtgcaatgtaacatcagagattttgagacacgggccagagctgca

SEQ ID NO: 34 - DNA, 4285 bp, synthetic construct
  source 1..4285: mol_type = other DNA
tcgcgcgtttcggtgatgacggtgaaaacctctgacacatgcagctcccggacgtcattgtcgatgctagcctgcgcgctcgctcgctcactgaggccgcccgggcaaagcccgggcgtcgggcgacctttggtcgcccggcctcagtgagcgagcgagcgcgcagagagggagtggataggcgccaagagcctagacttccttaagcgccagagtccacaagggcccagttaatcctcaacattcaaatgctgcccacaaaaccagcccctctgtgccctagccgcctcttttttccaagtgacagtagaactccaccaatccgcagctgaatggggtccgcctcttttccctgcctaaacagacaggaactcctgccaattgagggcgtcaccgctaaggctccgccccagcctgggctccacaaccaatgaagggtaatctcgacaaagagcaaggggtggggcgcgggcgcgcaggtgcagcagcacacaggctggtcgggagggcggggcgcgacgtctgccgtgcggggtcccggcatcggttgcgcgcgcgctccctcctctcggagagagggctgtggtaaaacccgtccggaaaccatggccgccgccgccgccgccgcgccgagcggaggaggaggaggaggcgaggaggagagactggaagaaaagtcagaagaccaggacctccagggcctcaaggacaaacccctcaagtttaaaaaggtgaagaaagataagaaagaagagaaagagggcaagcatgagcccgtgcagccatcagcccaccactctgctgagcccgcagaggcaggcaaagcagagacatcagaagggtcaggctccgccccggctgtgccggaagcttctgcctcccccaaacagcggcgctccatcatccgtgaccggggacccatgtatgatgaccccaccctgcctgaaggctggacacggaagcttaagcaaaggaaatctggccgctctgctgggaagtatgatgtgtatttgatcaatccccagggaaaagcctttcgctctaaagtggagttgattgcgtacttcgaaaaggtaggcgacacatccctggaccctaatgattttgacttcacggtaactgggagagggagcccctcccggcgagagcagaaaccacctaagaagcccaaatctcccaaagctccaggaactggcagaggccggggacgccccaaagggagcggcaccacgagacccaaggcggccacgtcagagggtgtgcaggtgaaaagggtcctggagaaaagtcctgggaagctccttgtcaagatgccttttcaaacttcgccagggggcaaggctgaggggggtggggccaccacatccacccaggtcatggtgatcaaacgccccggcaggaagcgaaaagctgaggccgaccctcaggccattcccaagaaacggggccgaaagccggggagtgtggtggcagccgctgccgccgaggccaaaaagaaagccgtgaaggagtcttctatccgatctgtgcaggagaccgtactccccatcaagaagcgcaagacccgggagacggtcagcatcgaggtcaaggaagtggtgaagcccctgctggtgtccaccctcggtgagaagagcgggaaaggactgaagacctgtaagagccctgggcggaaaagcaaggagagcagccccaaggggcgcagcagcagcgcctcctcaccccccaagaaggagcaccaccaccatcaccaccactcagagtccccaaaggcccccgtgccactgctcccacccctgcccccacctccacctgagcccgagagctccgaggaccccaccagcccccctgagccccaggacttgagcagcagcgtctgcaaagaggagaagatgcccagaggaggctcactggagagcgacggctgccccaaggagccagctaagactcagcccgcggttgccaccgccgccacggccgcagaaaagtacaaacaccgaggggagggagagcgcaaagacattgtttcatcctccatgccaaggccaaacagagaggagcctgtggacagccggacgcccgtgaccgagagagttagcgggagctccggcagttctggagaacaaaaactcatctcagaagaggatctgtgaacaagaataaaggcagctgttgtctcttctccttatgggtagggctctgacaaagcttcccatatcaccaggactgttaatatatttaaaaacaaaaggcaatttattaaggaaatttgtaccatttcagtaaacctgtctgaaccggcacaagatcggatctacgggttgttttataaagagtttgccttataaatttacataaaaatgtccgtttgtgtcttttgttgaggaacccctagtgatggagttggccactccctctctgcgcgctcgctcgctcactgaggccgggcgaccaaaggtcgcccgacgcccgggctttgcccgggcggcctcagtgagcgagcgagcgcgcagagagggagtggccatcattgtcacatgtgagcaaaaggccagcaaaaggccaggaaccgtaaaaaggccgcgttgctggcgtttttccataggctccgcccccctgacgagcatcacaaaaatcgacgctcaagtcagaggtggcgaaacccgacaggactataaagataccaggcgtttccccctggaagctccctcgtgcgctctcctgttccgaccctgccgcttaccggatacctgtccgcctttctcccttcgggaagcgtggcgctttctcatagctcacgctgtaggtatctcagttcggtgtaggtcgttcgctccaagctgggctgtgtgcacgaaccccccgttcagcccgaccgctgcgccttatccggtaactatcgtcttgagtccaacccggtaagacacgacttatcgccactggcagcagccactggtaacaggattagcagagcgaggtatgtaggcggtgctacagagttcttgaagtggtggcctaactacggctacactagaagaacagtatttggtatctgcgctctgctgaagccagttaccttcggaaaaagagttggtagctcttgatccggcaaacaaaccaccgctggtagcggtggtttttttgtttgcaagcagcagattacgcgcagaaaaaaaggatctcaagaagatcctttgatcttttctacggggtctgacgctcagtggaacgaaaactcacgttaagggattttggtcatgagattatcaaaaaggatcttcacctagatccttttaaattaaaaatgaagttttaaatcaagcccaatctgaataatgttacaaccaattaaccaattctgattagaaaaactcatcgagcatcaaatgaaactgcaatttattcatatcaggattatcaataccatatttttgaaaaagccgtttctgtaatgaaggagaaaactcaccgaggcagttccataggatggcaagatcctggtatcggtctgcgattccgactcgtccaacatcaatacaacctattaatttcccctcgtcaaaaataaggttatcaagtgagaaatcaccatgagtgacgactgaatccggtgagaatggcaaaagtttatgcatttctttccagacttgttcaacaggccagccattacgctcgtcatcaaaatcactcgcatcaaccaaaccgttattcattcgtgattgcgcctgagcgagacgaaatacgcgatcgctgttaaaaggacaattacaaacaggaatcgaatgcaaccggcgcaggaacactgccagcgcatcaacaatattttcacctgaatcaggatattcttctaatacctggaatgctgtttttccggggatcgcagtggtgagtaaccatgcatcatcaggagtacggataaaatgcttgatggtcggaagaggcataaattccgtcagccagtttagtctgaccatctcatctgtaacatcattggcaacgctacctttgccatgtttcagaaacaactctggcgcatcgggcttcccatacaagcgatagattgtcgcacctgattgcccgacattatcgcgagcccatttatacccatataaatcagcatccatgttggaatttaatcgcggcctcgacgtttcccgttgaatatggctcataacaccccttgtattactgtttatgtaagcagacagttttattgttcatgatgatatatttttatcttgtgcaatgtaacatcagagattttgagacacgggccagagctgca

SEQ ID NO: 35 - DNA, 4285 bp, synthetic construct
  source 1..4285: mol_type = other DNA
tcgcgcgtttcggtgatgacggtgaaaacctctgacacatgcagctcccggacgtcattgtcgatgctagcctgcgcgctcgctcgctcactgaggccgcccgggcaaagcccgggcgtcgggcgacctttggtcgcccggcctcagtgagcgagcgagcgcgcagagagggagtggataggcgccaagagcctagacttccttaagcgccagagtccacaagggcccagttaatcctcaacattcaaatgctgcccacaaaaccagcccctctgtgccctagccgcctcttttttccaagtgacagtagaactccaccaatccgcagctgaatggggtccgcctcttttccctgcctaaacagacaggaactcctgccaattgagggcgtcaccgctaaggctccgccccagcctgggctccacaaccaatgaagggtaatctcgacaaagagcaaggggtggggcgcgggcgcgcaggtgcagcagcacacaggctggtcgggagggcggggcgcgacgtctgccgtgcggggtcccggcatcggttgcgcgcgcgctccctcctctcggagagagggctgtggtaaaacccgtccggaaaccatggccgccgccgccgccgccgcgccgagcggaggaggaggaggaggcgaggaggagagactggaagaaaagtcagaagaccaggacctccagggcctcaaggacaaacccctcaagtttaaaaaggtgaagaaagataagaaagaagagaaagagggcaagcatgagcccgtgcagccatcagcccaccactctgctgagcccgcagaggcaggcaaagcagagacatcagaagggtcaggctccgccccggctgtgccggaagcttctgcctcccccaaacagcggcgctccatcatccgtgaccggggacccatgtatgatgaccccaccctgcctgaaggctggacacggaagcttaagcaaaggaaatctggccgctctgctgggaagtatgatgtgtatttgatcaatccccagggaaaagcctttcgctctaaagtggagttgattgcgtacttcgaaaaggtaggcgacacatccctggaccctaatgattttgacttcacggtaactgggagagggagcccctcccggcgagagcagaaaccacctaagaagcccaaatctcccaaagctccaggaactggcagaggccggggacgccccaaagggagcggcaccacgagacccaaggcggccacgtcagagggtgtgcaggtgaaaagggtcctggagaaaagtcctgggaagctccttgtcaagatgccttttcaaacttcgccagggggcaaggctgaggggggtggggccaccacatccacccaggtcatggtgatcaaacgccccggcaggaagcgaaaagctgaggccgaccctcaggccattcccaagaaacggggccgaaagccggggagtgtggtggcagccgctgccgccgaggccaaaaagaaagccgtgaaggagtcttctatccgatctgtgcaggagaccgtactccccatcaagaagcgcaagacccgggagacggtcagcatcgaggtcaaggaagtggtgaagcccctgctggtgtccaccctcggtgagaagagcgggaaaggactgaagacctgtaagagccctgggcggaaaagcaaggagagcagccccaaggggcgcagcagcagcgcctcctcaccccccaagaaggagcaccaccaccatcaccaccactcagagtccccaaaggcccccgtgccactgctcccacccctgcccccacctccacctgagcccgagagctccgaggaccccaccagcccccctgagccccaggacttgagcagcagcgtctgcaaagaggagaagatgcccagaggaggctcactggagagcgacggctgccccaaggagccagctaagactcagcccgcggttgccaccgccgccacggccgcagaaaagtacaaacaccgaggggagggagagcgcaaagacattgtttcatcctccatgccaaggccaaacagagaggagcctgtggacagccggacgcccgtgaccgagagagttagcgggagctccggcagttctggagaacaaaaactcatctcagaagaggatctgtgaacaagaataaaggcagctgttgtctcttctccttatgggtagggctctgacaaagcttcccatatcaccaggactgttaatatatttaaaaacaaaaggcaatttattaaggaaatttgtaccatttcagtaaacctgtctgaaccggcacaagttcggatctacgggttgttttataaagagtttgccttataaatttacataaaaatgtccgtttgtgtcttttgttgaggaacccctagtgatggagttggccactccctctctgcgcgctcgctcgctcactgaggccgggcgaccaaaggtcgcccgacgcccgggctttgcccgggcggcctcagtgagcgagcgagcgcgcagagagggagtggccatcattgtcacatgtgagcaaaaggccagcaaaaggccaggaaccgtaaaaaggccgcgttgctggcgtttttccataggctccgcccccctgacgagcatcacaaaaatcgacgctcaagtcagaggtggcgaaacccgacaggactataaagataccaggcgtttccccctggaagctccctcgtgcgctctcctgttccgaccctgccgcttaccggatacctgtccgcctttctcccttcgggaagcgtggcgctttctcatagctcacgctgtaggtatctcagttcggtgtaggtcgttcgctccaagctgggctgtgtgcacgaaccccccgttcagcccgaccgctgcgccttatccggtaactatcgtcttgagtccaacccggtaagacacgacttatcgccactggcagcagccactggtaacaggattagcagagcgaggtatgtaggcggtgctacagagttcttgaagtggtggcctaactacggctacactagaagaacagtatttggtatctgcgctctgctgaagccagttaccttcggaaaaagagttggtagctcttgatccggcaaacaaaccaccgctggtagcggtggtttttttgtttgcaagcagcagattacgcgcagaaaaaaaggatctcaagaagatcctttgatcttttctacggggtctgacgctcagtggaacgaaaactcacgttaagggattttggtcatgagattatcaaaaaggatcttcacctagatccttttaaattaaaaatgaagttttaaatcaagcccaatctgaataatgttacaaccaattaaccaattctgattagaaaaactcatcgagcatcaaatgaaactgcaatttattcatatcaggattatcaataccatatttttgaaaaagccgtttctgtaatgaaggagaaaactcaccgaggcagttccataggatggcaagatcctggtatcggtctgcgattccgactcgtccaacatcaatacaacctattaatttcccctcgtcaaaaataaggttatcaagtgagaaatcaccatgagtgacgactgaatccggtgagaatggcaaaagtttatgcatttctttccagacttgttcaacaggccagccattacgctcgtcatcaaaatcactcgcatcaaccaaaccgttattcattcgtgattgcgcctgagcgagacgaaatacgcgatcgctgttaaaaggacaattacaaacaggaatcgaatgcaaccggcgcaggaacactgccagcgcatcaacaatattttcacctgaatcaggatattcttctaatacctggaatgctgtttttccggggatcgcagtggtgagtaaccatgcatcatcaggagtacggataaaatgcttgatggtcggaagaggcataaattccgtcagccagtttagtctgaccatctcatctgtaacatcattggcaacgctacctttgccatgtttcagaaacaactctggcgcatcgggcttcccatacaagcgatagattgtcgcacctgattgcccgacattatcgcgagcccatttatacccatataaatcagcatccatgttggaatttaatcgcggcctcgacgtttcccgttgaatatggctcataacaccccttgtattactgtttatgtaagcagacagttttattgttcatgatgatatatttttatcttgtgcaatgtaacatcagagattttgagacacgggccagagctgca

SEQ ID NO: 36 - DNA, 4286 bp, synthetic construct
  source 1..4286: mol_type = other DNA
tcgcgcgtttcggtgatgacggtgaaaacctctgacacatgcagctcccggacgtcattgtcgatgctagcctgcgcgctcgctcgctcactgaggccgcccgggcaaagcccgggcgtcgggcgacctttggtcgcccggcctcagtgagcgagcgagcgcgcagagagggagtggataggcgccaagagcctagacttccttaagcgccagagtccacaagggcccagttaatcctcaacattcaaatgctgcccacaaaaccagcccctctgtgccctagccgcctcttttttccaagtgacagtagaactccaccaatccgcagctgaatggggtccgcctcttttccctgcctaaacagacaggaactcctgccaattgagggcgtcaccgctaaggctccgccccagcctgggctccacaaccaatgaagggtaatctcgacaaagagcaaggggtggggcgcgggcgcgcaggtgcagcagcacacaggctggtcgggagggcggggcgcgacgtctgccgtgcggggtcccggcatcggttgcgcgcgcgctccctcctctcggagagagggctgtggtaaaacccgtccggaaaccatggccgccgccgccgccgccgcgccgagcggaggaggaggaggaggcgaggaggagagactggaagaaaagtcagaagaccaggacctccagggcctcaaggacaaacccctcaagtttaaaaaggtgaagaaagataagaaagaagagaaagagggcaagcatgagcccgtgcagccatcagcccaccactctgctgagcccgcagaggcaggcaaagcagagacatcagaagggtcaggctccgccccggctgtgccggaagcttctgcctcccccaaacagcggcgctccatcatccgtgaccggggacccatgtatgatgaccccaccctgcctgaaggctggacacggaagcttaagcaaaggaaatctggccgctctgctgggaagtatgatgtgtatttgatcaatccccagggaaaagcctttcgctctaaagtggagttgattgcgtacttcgaaaaggtaggcgacacatccctggaccctaatgattttgacttcacggtaactgggagagggagcccctcccggcgagagcagaaaccacctaagaagcccaaatctcccaaagctccaggaactggcagaggccggggacgccccaaagggagcggcaccacgagacccaaggcggccacgtcagagggtgtgcaggtgaaaagggtcctggagaaaagtcctgggaagctccttgtcaagatgccttttcaaacttcgccagggggcaaggctgaggggggtggggccaccacatccacccaggtcatggtgatcaaacgccccggcaggaagcgaaaagctgaggccgaccctcaggccattcccaagaaacggggccgaaagccggggagtgtggtggcagccgctgccgccgaggccaaaaagaaagccgtgaaggagtcttctatccgatctgtgcaggagaccgtactccccatcaagaagcgcaagacccgggagacggtcagcatcgaggtcaaggaagtggtgaagcccctgctggtgtccaccctcggtgagaagagcgggaaaggactgaagacctgtaagagccctgggcggaaaagcaaggagagcagccccaaggggcgcagcagcagcgcctcctcaccccccaagaaggagcaccaccaccatcaccaccactcagagtccccaaaggcccccgtgccactgctcccacccctgcccccacctccacctgagcccgagagctccgaggaccccaccagcccccctgagccccaggacttgagcagcagcgtctgcaaagaggagaagatgcccagaggaggctcactggagagcgacggctgccccaaggagccagctaagactcagcccgcggttgccaccgccgccacggccgcagaaaagtacaaacaccgaggggagggagagcgcaaagacattgtttcatcctccatgccaaggccaaacagagaggagcctgtggacagccggacgcccgtgaccgagagagttagcgggagctccggcagttctggagaacaaaaactcatctcagaagaggatctgtgaacaagaataaaggcagctgttgtctcttctccttatgggtagggctctgacaaagcttcccatatcaccaggactgttaatatatttaaaaacaaaaggcaatttattaaggaaatttgtaccatttcagtaaacctgtctgaaccggacaaggatgaatctttgttactggttttataaagagtttgccttataaatttacataaaaatgtccgtttgtgtcttttgttgaggaacccctagtgatggagttggccactccctctctgcgcgctcgctcgctcactgaggccgggcgaccaaaggtcgcccgacgcccgggctttgcccgggcggcctcagtgagcgagcgagcgcgcagagagggagtggccatcattgtcacatgtgagcaaaaggccagcaaaaggccaggaaccgtaaaaaggccgcgttgctggcgtttttccataggctccgcccccctgacgagcatcacaaaaatcgacgctcaagtcagaggtggcgaaacccgacaggactataaagataccaggcgtttccccctggaagctccctcgtgcgctctcctgttccgaccctgccgcttaccggatacctgtccgcctttctcccttcgggaagcgtggcgctttctcatagctcacgctgtaggtatctcagttcggtgtaggtcgttcgctccaagctgggctgtgtgcacgaaccccccgttcagcccgaccgctgcgccttatccggtaactatcgtcttgagtccaacccggtaagacacgacttatcgccactggcagcagccactggtaacaggattagcagagcgaggtatgtaggcggtgctacagagttcttgaagtggtggcctaactacggctacactagaagaacagtatttggtatctgcgctctgctgaagccagttaccttcggaaaaagagttggtagctcttgatccggcaaacaaaccaccgctggtagcggtggtttttttgtttgcaagcagcagattacgcgcagaaaaaaaggatctcaagaagatcctttgatcttttctacggggtctgacgctcagtggaacgaaaactcacgttaagggattttggtcatgagattatcaaaaaggatcttcacctagatccttttaaattaaaaatgaagttttaaatcaagcccaatctgaataatgttacaaccaattaaccaattctgattagaaaaactcatcgagcatcaaatgaaactgcaatttattcatatcaggattatcaataccatatttttgaaaaagccgtttctgtaatgaaggagaaaactcaccgaggcagttccataggatggcaagatcctggtatcggtctgcgattccgactcgtccaacatcaatacaacctattaatttcccctcgtcaaaaataaggttatcaagtgagaaatcaccatgagtgacgactgaatccggtgagaatggcaaaagtttatgcatttctttccagacttgttcaacaggccagccattacgctcgtcatcaaaatcactcgcatcaaccaaaccgttattcattcgtgattgcgcctgagcgagacgaaatacgcgatcgctgttaaaaggacaattacaaacaggaatcgaatgcaaccggcgcaggaacactgccagcgcatcaacaatattttcacctgaatcaggatattcttctaatacctggaatgctgtttttccggggatcgcagtggtgagtaaccatgcatcatcaggagtacggataaaatgcttgatggtcggaagaggcataaattccgtcagccagtttagtctgaccatctcatctgtaacatcattggcaacgctacctttgccatgtttcagaaacaactctggcgcatcgggcttcccatacaagcgatagattgtcgcacctgattgcccgacattatcgcgagcccatttatacccatataaatcagcatccatgttggaatttaatcgcggcctcgacgtttcccgttgaatatggctcataacaccccttgtattactgtttatgtaagcagacagttttattgttcatgatgatatatttttatcttgtgcaatgtaacatcagagattttgagacacgggccagagctgca

SEQ ID NO: 37 - DNA, 4285 bp, synthetic construct
  source 1..4285: mol_type = other DNA
tcgcgcgtttcggtgatgacggtgaaaacctctgacacatgcagctcccggacgtcattgtcgatgctagcctgcgcgctcgctcgctcactgaggccgcccgggcaaagcccgggcgtcgggcgacctttggtcgcccggcctcagtgagcgagcgagcgcgcagagagggagtggataggcgccaagagcctagacttccttaagcgccagagtccacaagggcccagttaatcctcaacattcaaatgctgcccacaaaaccagcccctctgtgccctagccgcctcttttttccaagtgacagtagaactccaccaatccgcagctgaatggggtccgcctcttttccctgcctaaacagacaggaactcctgccaattgagggcgtcaccgctaaggctccgccccagcctgggctccacaaccaatgaagggtaatctcgacaaagagcaaggggtggggcgcgggcgcgcaggtgcagcagcacacaggctggtcgggagggcggggcgcgacgtctgccgtgcggggtcccggcatcggttgcgcgcgcgctccctcctctcggagagagggctgtggtaaaacccgtccggaaaccatggccgccgccgccgccgccgcgccgagcggaggaggaggaggaggcgaggaggagagactggaagaaaagtcagaagaccaggacctccagggcctcaaggacaaacccctcaagtttaaaaaggtgaagaaagataagaaagaagagaaagagggcaagcatgagcccgtgcagccatcagcccaccactctgctgagcccgcagaggcaggcaaagcagagacatcagaagggtcaggctccgccccggctgtgccggaagcttctgcctcccccaaacagcggcgctccatcatccgtgaccggggacccatgtatgatgaccccaccctgcctgaaggctggacacggaagcttaagcaaaggaaatctggccgctctgctgggaagtatgatgtgtatttgatcaatccccagggaaaagcctttcgctctaaagtggagttgattgcgtacttcgaaaaggtaggcgacacatccctggaccctaatgattttgacttcacggtaactgggagagggagcccctcccggcgagagcagaaaccacctaagaagcccaaatctcccaaagctccaggaactggcagaggccggggacgccccaaagggagcggcaccacgagacccaaggcggccacgtcagagggtgtgcaggtgaaaagggtcctggagaaaagtcctgggaagctccttgtcaagatgccttttcaaacttcgccagggggcaaggctgaggggggtggggccaccacatccacccaggtcatggtgatcaaacgccccggcaggaagcgaaaagctgaggccgaccctcaggccattcccaagaaacggggccgaaagccggggagtgtggtggcagccgctgccgccgaggccaaaaagaaagccgtgaaggagtcttctatccgatctgtgcaggagaccgtactccccatcaagaagcgcaagacccgggagacggtcagcatcgaggtcaaggaagtggtgaagcccctgctggtgtccaccctcggtgagaagagcgggaaaggactgaagacctgtaagagccctgggcggaaaagcaaggagagcagccccaaggggcgcagcagcagcgcctcctcaccccccaagaaggagcaccaccaccatcaccaccactcagagtccccaaaggcccccgtgccactgctcccacccctgcccccacctccacctgagcccgagagctccgaggaccccaccagcccccctgagccccaggacttgagcagcagcgtctgcaaagaggagaagatgcccagaggaggctcactggagagcgacggctgccccaaggagccagctaagactcagcccgcggttgccaccgccgccacggccgcagaaaagtacaaacaccgaggggagggagagcgcaaagacattgtttcatcctccatgccaaggccaaacagagaggagcctgtggacagccggacgcccgtgaccgagagagttagcgggagctccggcagttctggagaacaaaaactcatctcagaagaggatctgtgaacaagaataaaggcagctgttgtctcttctccttatgggtagggctctgacaaagcttcccatatcaccaggactgttaatatatttaaaaacaaaaggcaatttattaaggaaatttgtaccatttcagtaaacctgtctgaaccgggaggctcagaatggctcaggaggttttataaagagtttgccttataaatttacataaaaatgtccgtttgtgtcttttgttgaggaacccctagtgatggagttggccactccctctctgcgcgctcgctcgctcactgaggccgggcgaccaaaggtcgcccgacgcccgggctttgcccgggcggcctcagtgagcgagcgagcgcgcagagagggagtggccatcattgtcacatgtgagcaaaaggccagcaaaaggccaggaaccgtaaaaaggccgcgttgctggcgtttttccataggctccgcccccctgacgagcatcacaaaaatcgacgctcaagtcagaggtggcgaaacccgacaggactataaagataccaggcgtttccccctggaagctccctcgtgcgctctcctgttccgaccctgccgcttaccggatacctgtccgcctttctcccttcgggaagcgtggcgctttctcatagctcacgctgtaggtatctcagttcggtgtaggtcgttcgctccaagctgggctgtgtgcacgaaccccccgttcagcccgaccgctgcgccttatccggtaactatcgtcttgagtccaacccggtaagacacgacttatcgccactggcagcagccactggtaacaggattagcagagcgaggtatgtaggcggtgctacagagttcttgaagtggtggcctaactacggctacactagaagaacagtatttggtatctgcgctctgctgaagccagttaccttcggaaaaagagttggtagctcttgatccggcaaacaaaccaccgctggtagcggtggtttttttgtttgcaagcagcagattacgcgcagaaaaaaaggatctcaagaagatcctttgatcttttctacggggtctgacgctcagtggaacgaaaactcacgttaagggattttggtcatgagattatcaaaaaggatcttcacctagatccttttaaattaaaaatgaagttttaaatcaagcccaatctgaataatgttacaaccaattaaccaattctgattagaaaaactcatcgagcatcaaatgaaactgcaatttattcatatcaggattatcaataccatatttttgaaaaagccgtttctgtaatgaaggagaaaactcaccgaggcagttccataggatggcaagatcctggtatcggtctgcgattccgactcgtccaacatcaatacaacctattaatttcccctcgtcaaaaataaggttatcaagtgagaaatcaccatgagtgacgactgaatccggtgagaatggcaaaagtttatgcatttctttccagacttgttcaacaggccagccattacgctcgtcatcaaaatcactcgcatcaaccaaaccgttattcattcgtgattgcgcctgagcgagacgaaatacgcgatcgctgttaaaaggacaattacaaacaggaatcgaatgcaaccggcgcaggaacactgccagcgcatcaacaatattttcacctgaatcaggatattcttctaatacctggaatgctgtttttccggggatcgcagtggtgagtaaccatgcatcatcaggagtacggataaaatgcttgatggtcggaagaggcataaattccgtcagccagtttagtctgaccatctcatctgtaacatcattggcaacgctacctttgccatgtttcagaaacaactctggcgcatcgggcttcccatacaagcgatagattgtcgcacctgattgcccgacattatcgcgagcccatttatacccatataaatcagcatccatgttggaatttaatcgcggcctcgacgtttcccgttgaatatggctcataacaccccttgtattactgtttatgtaagcagacagttttattgttcatgatgatatatttttatcttgtgcaatgtaacatcagagattttgagacacgggccagagctgca

SEQ ID NO: 38 - DNA, 2205 bp, synthetic construct
  source 1..2205: mol_type = other DNA
ataggcgccaagagcctagacttccttaagcgccagagtccacaagggcccagttaatcctcaacattcaaatgctgcccacaaaaccagcccctctgtgccctagccgcctcttttttccaagtgacagtagaactccaccaatccgcagctgaatggggtccgcctcttttccctgcctaaacagacaggaactcctgccaattgagggcgtcaccgctaaggctccgccccagcctgggctccacaaccaatgaagggtaatctcgacaaagagcaaggggtggggcgcgggcgcgcaggtgcagcagcacacaggctggtcgggagggcggggcgcgacgtctgccgtgcggggtcccggcatcggttgcgcgcgcgctccctcctctcggagagagggctgtggtaaaacccgtccggaaaccatggccgccgccgccgccgccgcgccgagcggaggaggaggaggaggcgaggaggagagactggaagaaaagtcagaagaccaggacctccagggcctcaaggacaaacccctcaagtttaaaaaggtgaagaaagataagaaagaagagaaagagggcaagcatgagcccgtgcagccatcagcccaccactctgctgagcccgcagaggcaggcaaagcagagacatcagaagggtcaggctccgccccggctgtgccggaagcttctgcctcccccaaacagcggcgctccatcatccgtgaccggggacccatgtatgatgaccccaccctgcctgaaggctggacacggaagcttaagcaaaggaaatctggccgctctgctgggaagtatgatgtgtatttgatcaatccccagggaaaagcctttcgctctaaagtggagttgattgcgtacttcgaaaaggtaggcgacacatccctggaccctaatgattttgacttcacggtaactgggagagggagcccctcccggcgagagcagaaaccacctaagaagcccaaatctcccaaagctccaggaactggcagaggccggggacgccccaaagggagcggcaccacgagacccaaggcggccacgtcagagggtgtgcaggtgaaaagggtcctggagaaaagtcctgggaagctccttgtcaagatgccttttcaaacttcgccagggggcaaggctgaggggggtggggccaccacatccacccaggtcatggtgatcaaacgccccggcaggaagcgaaaagctgaggccgaccctcaggccattcccaagaaacggggccgaaagccggggagtgtggtggcagccgctgccgccgaggccaaaaagaaagccgtgaaggagtcttctatccgatctgtgcaggagaccgtactccccatcaagaagcgcaagacccgggagacggtcagcatcgaggtcaaggaagtggtgaagcccctgctggtgtccaccctcggtgagaagagcgggaaaggactgaagacctgtaagagccctgggcggaaaagcaaggagagcagccccaaggggcgcagcagcagcgcctcctcaccccccaagaaggagcaccaccaccatcaccaccactcagagtccccaaaggcccccgtgccactgctcccacccctgcccccacctccacctgagcccgagagctccgaggaccccaccagcccccctgagccccaggacttgagcagcagcgtctgcaaagaggagaagatgcccagaggaggctcactggagagcgacggctgccccaaggagccagctaagactcagcccgcggttgccaccgccgccacggccgcagaaaagtacaaacaccgaggggagggagagcgcaaagacattgtttcatcctccatgccaaggccaaacagagaggagcctgtggacagccggacgcccgtgaccgagagagttagcgggagctccggcagttctggagaacaaaaactcatctcagaagaggatctgtgaacaagaataaaggcagctgttgtctcttctccttatgggtagggctctgacaaagcttcccatatcaccaggactgttaatatatttaaaaacaaaaggcaatttattaaggaaatttgtaccatttcagtaaacctgtctgaaccggagagaccgagagagggtctcagttttataaagagtttgccttataaatttacataaaaatgtccgtttgtgtcttttgttg

SEQ ID NO: 39 - DNA, 2303 bp, synthetic construct
  source 1..2303: mol_type = other DNA
ataggcgccaagagcctagacttccttaagcgccagagtccacaagggcccagttaatcctcaacattcaaatgctgcccacaaaaccagcccctctgtgccctagccgcctcttttttccaagtgacagtagaactccaccaatccgcagctgaatggggtccgcctcttttccctgcctaaacagacaggaactcctgccaattgagggcgtcaccgctaaggctccgccccagcctgggctccacaaccaatgaagggtaatctcgacaaagagcaaggggtggggcgcgggcgcgcaggtgcagcagcacacaggctggtcgggagggcggggcgcgacgtctgccgtgcggggtcccggcatcggttgcgcgcgcgctccctcctctcggagagagggctgtggtaaaacccgtccggaaaccatggccgccgccgccgccgccgcgccgagcggaggaggaggaggaggcgaggaggagagactggaagaaaagtcagaagaccaggacctccagggcctcaaggacaaacccctcaagtttaaaaaggtgaagaaagataagaaagaagagaaagagggcaagcatgagcccgtgcagccatcagcccaccactctgctgagcccgcagaggcaggcaaagcagagacatcagaagggtcaggctccgccccggctgtgccggaagcttctgcctcccccaaacagcggcgctccatcatccgtgaccggggacccatgtatgatgaccccaccctgcctgaaggctggacacggaagcttaagcaaaggaaatctggccgctctgctgggaagtatgatgtgtatttgatcaatccccagggaaaagcctttcgctctaaagtggagttgattgcgtacttcgaaaaggtaggcgacacatccctggaccctaatgattttgacttcacggtaactgggagagggagcccctcccggcgagagcagaaaccacctaagaagcccaaatctcccaaagctccaggaactggcagaggccggggacgccccaaagggagcggcaccacgagacccaaggcggccacgtcagagggtgtgcaggtgaaaagggtcctggagaaaagtcctgggaagctccttgtcaagatgccttttcaaacttcgccagggggcaaggctgaggggggtggggccaccacatccacccaggtcatggtgatcaaacgccccggcaggaagcgaaaagctgaggccgaccctcaggccattcccaagaaacggggccgaaagccggggagtgtggtggcagccgctgccgccgaggccaaaaagaaagccgtgaaggagtcttctatccgatctgtgcaggagaccgtactccccatcaagaagcgcaagacccgggagacggtcagcatcgaggtcaaggaagtggtgaagcccctgctggtgtccaccctcggtgagaagagcgggaaaggactgaagacctgtaagagccctgggcggaaaagcaaggagagcagccccaaggggcgcagcagcagcgcctcctcaccccccaagaaggagcaccaccaccatcaccaccactcagagtccccaaaggcccccgtgccactgctcccacccctgcccccacctccacctgagcccgagagctccgaggaccccaccagcccccctgagccccaggacttgagcagcagcgtctgcaaagaggagaagatgcccagaggaggctcactggagagcgacggctgccccaaggagccagctaagactcagcccgcggttgccaccgccgccacggccgcagaaaagtacaaacaccgaggggagggagagcgcaaagacattgtttcatcctccatgccaaggccaaacagagaggagcctgtggacagccggacgcccgtgaccgagagagttagcgggagctccggcagttctggagaacaaaaactcatctcagaagaggatctgtgaacaagaataaaggcagctgttgtctcttctccttatgggtagggctctgacaaagcttcccatatcaccaggactgttaatatatttaaaaacaaaaggcaatttattaaggaaatttgtaccagtgaattctaccagtgccatagtacctgtatacgtttcaaaaactcccttctttcctcccgtctacaccccccccccactgaatccaaacaccattgtcacactccacctgtaacctatttattaatgcccttttaacattgcactatataaagagtttgccttataaatttacataaaaatgtccgtttgtgtcttttgttg